European Patent Specification EP 3 456 192 B1, published September 3, 2025. Title: Antibody producing non-human mammals. Applicant: Merus N.V. Application EP12175544.1. The sequence listing filed with the application follows.

SEQUENCE LISTING (101 sequences)

SEQ ID NO: 1 - DNA, 20 bp, Artificial
  primer
ccctttccaatctttatggg

SEQ ID NO: 2 - DNA, 23 bp, Artificial
  primer
aggtggattggtgtctttttctc

SEQ ID NO: 3 - DNA, 22 bp, Artificial
  primer
gtcatgtcggcgaccctacgcc

SEQ ID NO: 4 - DNA, 20 bp, Artificial
  primer
tgccagggggaagaccgatg

SEQ ID NO: 5 - DNA, 38 bp, Artificial
  primer
gccggccatggccgaggtrmagcttcaggagtcaggac

SEQ ID NO: 6 - DNA, 38 bp, Artificial
  primer
gccggccatggccgaggtscagctkcagcagtcaggac

SEQ ID NO: 7 - DNA, 36 bp, Artificial
  primer
gccggccatggcccaggtgcagctgaagsastcagg

SEQ ID NO: 8 - DNA, 38 bp, Artificial
  primer
gccggccatggccgaggtgcagcttcaggagtcsggac

SEQ ID NO: 9 - DNA, 38 bp, Artificial
  primer
gccggccatggccgargtccagctgcaacagtcyggac

SEQ ID NO: 10 - DNA, 36 bp, Artificial
  primer
gccggccatggcccaggtccagctkcagcaatctgg

SEQ ID NO: 11 - DNA, 36 bp, Artificial
  primer
gccggccatggcccagstbcagctgcagcagtctgg

SEQ ID NO: 12 - DNA, 38 bp, Artificial
  primer
gccggccatggcccaggtycagctgcagcagtctggrc

SEQ ID NO: 13 - DNA, 36 bp, Artificial
  primer
gccggccatggcccaggtycagctycagcagtctgg

SEQ ID NO: 14 - DNA, 39 bp, Artificial
  primer
gccggccatggccgaggtccarctgcaacaatctggacc

SEQ ID NO: 15 - DNA, 37 bp, Artificial
  primer
gccggccatggcccaggtccacgtgaagcagtctggg

SEQ ID NO: 16 - DNA, 35 bp, Artificial
  primer
gccggccatggccgaggtgaasstggtggaatctg

SEQ ID NO: 17 - DNA, 35 bp, Artificial
  primer
gccggccatggccgavgtgaagytggtggagtctg

SEQ ID NO: 18 - DNA, 38 bp, Artificial
  primer
gccggccatggccgaggtgcagskggtggagtctgggg

SEQ ID NO: 19 - DNA, 37 bp, Artificial
  primer
gccggccatggccgakgtgcamctggtggagtctggg

SEQ ID NO: 20 - DNA, 36 bp, Artificial
  primer
gccggccatggccgaggtgaagctgatggartctgg

SEQ ID NO: 21 - DNA, 38 bp, Artificial
  primer
gccggccatggccgaggtgcarcttgttgagtctggtg

SEQ ID NO: 22 - DNA, 37 bp, Artificial
  primer
gccggccatggccgargtraagcttctcgagtctgga

SEQ ID NO: 23 - DNA, 36 bp, Artificial
  primer
gccggccatggccgaagtgaarsttgaggagtctgg

SEQ ID NO: 24 - DNA, 37 bp, Artificial
  primer
gccggccatggccgaagtgatgctggtggagtctggg

SEQ ID NO: 25 - DNA, 38 bp, Artificial
  primer
gccggccatggcccaggttactctraaagwgtstggcc

SEQ ID NO: 26 - DNA, 36 bp, Artificial
  primer
gccggccatggcccaggtccaactvcagcarcctgg

SEQ ID NO: 27 - DNA, 35 bp, Artificial
  primer
gccggccatggcccaggtycarctgcagcagtctg

SEQ ID NO: 28 - DNA, 36 bp, Artificial
  primer
gccggccatggccgatgtgaacttggaagtgtctgg

SEQ ID NO: 29 - DNA, 36 bp, Artificial
  primer
gccggccatggccgaggtgaaggtcatcgagtctgg

SEQ ID NO: 30 - DNA, 45 bp, Artificial
  primer
  misc_feature (44)..(44): n is a, c, g, or t
cagtcacagatcctcgcgaattggcccagccggccatggccsang

SEQ ID NO: 31 - DNA, 45 bp, Artificial
  primer
  misc_feature (44)..(44): n is a, c, g, or t
cagtcacagatcctcgcgaattggcccagccggccatggccsanc

SEQ ID NO: 32 - DNA, 37 bp, Artificial
  primer
gggggtgtcgttttggctgaggagacggtgaccgtgg

SEQ ID NO: 33 - DNA, 37 bp, Artificial
  primer
gggggtgtcgttttggctgaggagactgtgagagtgg

SEQ ID NO: 34 - DNA, 37 bp, Artificial
  primer
gggggtgtcgttttggctgcagagacagtgaccagag

SEQ ID NO: 35 - DNA, 37 bp, Artificial
  primer
gggggtgtcgttttggctgaggagacggtgactgagg

SEQ ID NO: 36 - DNA, 37 bp, Artificial; identical to SEQ ID NO: 32
  primer

SEQ ID NO: 37 - DNA, 37 bp, Artificial
  primer
gggggtgtcgttttggctgaggagacggtgacagtgg

SEQ ID NO: 38 - DNA, 37 bp, Artificial
  primer
gggggtgtcgttttggctgaggagacggtgaccagag

SEQ ID NO: 39 - DNA, 37 bp, Artificial
  primer
gggggtgtcgttttggctgaggagacggtgaccgagg

SEQ ID NO: 40 - protein, 15 aa, Artificial
  CDR3
HGAYYTYDEKAWFAY

SEQ ID NO: 41 - protein, 15 aa, Artificial
  CDR3
HGAFYTYDEKPWFAY

SEQ ID NO: 42 - protein, 15 aa, Artificial
  CDR3
HISYYRYDEEVSFAY

SEQ ID NO: 43 - protein, 7 aa, Artificial
  CDR3
GWRAFAY

SEQ ID NO: 44 - protein, 10 aa, Artificial
  CDR3
DRGNYYGMDY

SEQ ID NO: 45 - protein, 12 aa, Artificial
  CDR3
LGDYYVDWFFAV

SEQ ID NO: 46 - protein, 8 aa, Artificial
  CDR3
NFPAWFAF

SEQ ID NO: 47 - protein, 17 aa, Artificial
  CDR3
SFTPVPFYYGYDWYFDV

SEQ ID NO: 48 - protein, 9 aa, Artificial
  CDR3
SDYDWYFDV

SEQ ID NO: 49 - protein, 10 aa, Artificial
  CDR3
DSKWAYYFDY

SEQ ID NO: 50 - protein, 10 aa, Artificial
  CDR3
GDYTGYGMDY

SEQ ID NO: 51 - protein, 10 aa, Artificial
  CDR3
GGYDGYWFPY

SEQ ID NO: 52 - protein, 15 aa, Artificial
  epitope IGKV1-39
DIQMTQSPSSLSASV

SEQ ID NO: 53 - protein, 15 aa, Artificial
  epitope IGKV1-39
MTQSPSSLSASVGDR

SEQ ID NO: 54 - protein, 15 aa, Artificial
  epitope IGKV1-39
SPSSLSASVGDRVTI

SEQ ID NO: 55 - protein, 15 aa, Artificial
  epitope IGKV1-39
SLSASVGDRVTITCR

SEQ ID NO: 56 - protein, 15 aa, Artificial
  Epitope IGKV1-39
ASVGDRVTITCRASQ

SEQ ID NO: 57 - protein, 15 aa, Artificial
  Epitope IGKV1-39
GDRVTITCRASQSIS

SEQ ID NO: 58 - protein, 15 aa, Artificial
  Epitope IGKV1-39
VTITCRASQSISSYL

SEQ ID NO: 59 - protein, 15 aa, Artificial
  Epitope IGKV1-39
TCRASQSISSYLNWY

SEQ ID NO: 60 - protein, 15 aa, Artificial
  Epitope IGKV1-39
ASQSISSYLNWYQQK

SEQ ID NO: 61 - protein, 15 aa, Artificial
  Epitope IGKV1-39
SISSYLNWYQQKPGK

SEQ ID NO: 62 - protein, 15 aa, Artificial
  Epitope IGKV1-39
SYLNWYQQKPGKAPK

SEQ ID NO: 63 - protein, 15 aa, Artificial
  Epitope IGKV1-39
NWYQQKPGKAPKLLI

SEQ ID NO: 64 - protein, 15 aa, Artificial
  Epitope IGKV1-39
QQKPGKAPKLLIYAA

SEQ ID NO: 65 - protein, 15 aa, Artificial
  Epitope IGKV1-39
PGKAPKLLIYAASSL

SEQ ID NO: 66 - protein, 15 aa, Artificial
  Epitope IGKV1-39
APKLLIYAASSLQSG

SEQ ID NO: 67 - protein, 15 aa, Artificial
  Epitope IGKV1-39
LLIYAASSLQSGVPS

SEQ ID NO: 68 - protein, 15 aa, Artificial
  Epitope IGKV1-39
YAASSLQSGVPSRFS

SEQ ID NO: 69 - protein, 15 aa, Artificial
  Epitope IGKV1-39
SSLQSGVPSRFSGSG

SEQ ID NO: 70 - protein, 15 aa, Artificial
  Epitope IGKV1-39
QSGVPSRFSGSGSGT

SEQ ID NO: 71 - protein, 15 aa, Artificial
  Epitope IGKV1-39
VPSRFSGSGSGTDFT

SEQ ID NO: 72 - protein, 15 aa, Artificial
  Epitope IGKV1-39
RFSGSGSGTDFTLTI

SEQ ID NO: 73 - protein, 15 aa, Artificial
  Epitope IGKV1-39
GSGSGTDFTLTISSL

SEQ ID NO: 74 - protein, 15 aa, Artificial
  Epitope IGKV1-39
SGTDFTLTISSLQPE

SEQ ID NO: 75 - protein, 15 aa, Artificial
  Epitope IGKV1-39
DFTLTISSLQPEDFA

SEQ ID NO: 76 - protein, 15 aa, Artificial
  Epitope IGKV1-39
LTISSLQPEDFATYY

SEQ ID NO: 77 - protein, 15 aa, Artificial
  Epitope IGKV1-39
SSLQPEDFATYYCQQ

SEQ ID NO: 78 - protein, 15 aa, Artificial
  Epitope IGKV1-39
QPEDFATYYCQQSYS

SEQ ID NO: 79 - protein, 15 aa, Artificial
  Epitope IGKV1-39
DFATYYCQQSYSTPP

SEQ ID NO: 80 - protein, 15 aa, Artificial
  Epitope IGKV1-39
TYYCQQSYSTPPTFG

SEQ ID NO: 81 - protein, 15 aa, Artificial
  Epitope IGKV1-39
CQQSYSTPPTFGQGT

SEQ ID NO: 82 - protein, 15 aa, Artificial
  Epitope IGKV1-39
SYSTPPTFGQGTKVE

SEQ ID NO: 83 - protein, 14 aa, Artificial
  Epitope IGKV1-39
TPPTFGQGTKVEIK

SEQ ID NO: 84 - DNA, 321 bp, Homo sapiens
  CDS (1)..(321)
gacatccagatgacccagagccccagcagcctgagcgccagcgtgggcgacagagtgaccatcacctgcagagccagccagagcatcagcagctacctgaactggtatcagcagaagcccggcaaggcccccaagctgctgatctacgccgccagctccctgcagagcggcgtgcccagcagattcagcggcagcggctccggcaccgacttcaccctgaccatcagcagcctgcagcccgaggacttcgccacctactactgccagcagagctacagcaccccccccaccttcggccagggcaccaaggtggagatcaag

SEQ ID NO: 85 - protein, 107 aa, Homo sapiens
DIQMTQSPSSLSASVGDRVTITCRASQSISSYLNWYQQKPGKAPKLLIYAASSLQSGVPSRFSGSGSGTDFTLTISSLQPEDFATYYCQQSYSTPPTFGQGTKVEIK

SEQ ID NO: 86 - DNA, 330 bp, Homo sapiens
  CDS (1)..(330)
cagtctgccctgacccagcccgcctctgtgtctggcagccctggccagagcatcaccatcagctgcaccggcaccagcagcgacgtgggcggctacaactacgtgtcctggtatcagcagcaccccggcaaggcccccaagctgatgatctacgaggtgtccaacagacccagcggcgtgagcaacagattcagcggcagcaagagcggcaacaccgccagcctgaccatcagcggcctccaggctgaggacgaggccgactactactgcagcagctacaccagcagctccaccctggtgtttggcggcggaacaaagctgaccgtgctg

SEQ ID NO: 87 - protein, 110 aa, Homo sapiens
QSALTQPASVSGSPGQSITISCTGTSSDVGGYNYVSWYQQHPGKAPKLMIYEVSNRPSGVSNRFSGSKSGNTASLTISGLQAEDEADYYCSSYTSSSTLVFGGGTKLTVL

SEQ ID NO: 88 - DNA, 321 bp, Rattus norvegicus
  CDS (1)..(321)
agagccgacgccgctcccaccgtgtccatcttcccccccagcatggaacagctgacctctggcggagccaccgtggtctgcttcgtgaacaacttctaccccagagacatcagcgtgaagtggaagatcgacggcagcgagcagagggacggcgtgctggacagcgtgaccgaccaggacagcaaggactccacctacagcatgagcagcaccctgagcctgaccaaggtggagtacgagaggcacaacctgtacacctgcgaggtggtgcacaagaccagctccagccccgtggtcaagtccttcaaccggaacgagtgt

SEQ ID NO: 89 - protein, 107 aa, Rattus norvegicus
RADAAPTVSIFPPSMEQLTSGGATVVCFVNNFYPRDISVKWKIDGSEQRDGVLDSVTDQDSKDSTYSMSSTLSLTKVEYERHNLYTCEVVHKTSSSPVVKSFNRNEC

SEQ ID NO: 90 - DNA, 865 bp, Artificial
  IGKV1-39/J-Ck
ggtaccgcggccgccaccatggacatgagagtgcccgcccagctcctggggctcctgctactctggctccgaggtaaggatggagaacactaggaatttactcagccagtgtgctcagtactgactggaacttcagggaagttctctgataacatgattaatagtaagaatatttgtttttatgtttccaatctcaggtgccagatgtgacatccagatgacccagagccccagcagcctgagcgccagcgtgggcgacagagtgaccatcacctgcagagccagccagagcatcagcagctacctgaactggtatcagcagaagcccggcaaggcccccaagctgctgatctacgccgccagctccctgcagagcggcgtgcccagcagattcagcggcagcggctccggcaccgacttcaccctgaccatcagcagcctgcagcccgaggacttcgccacctactactgccagcagagctacagcaccccccccaccttcggccagggcaccaaggtggagatcaagagagccgacgccgctcccaccgtgtccatcttcccccccagcatggaacagctgacctctggcggagccaccgtggtctgcttcgtgaacaacttctaccccagagacatcagcgtgaagtggaagatcgacggcagcgagcagagggacggcgtgctggacagcgtgaccgaccaggacagcaaggactccacctacagcatgagcagcaccctgagcctgaccaaggtggagtacgagaggcacaacctgtacacctgcgaggtggtgcacaagaccagctccagccccgtggtcaagtccttcaaccggaacgagtgttgagctagcgagctc

SEQ ID NO: 91 - DNA, 874 bp, Artificial
  IGLV2-14/J-Ck
ggtaccgcggccgccaccatggacatgagagtgcccgcccagctcctggggctcctgctactctggctccgaggtaaggatggagaacactaggaatttactcagccagtgtgctcagtactgactggaacttcagggaagttctctgataacatgattaatagtaagaatatttgtttttatgtttccaatctcaggtgccagatgtcagtctgccctgacccagcccgcctctgtgtctggcagccctggccagagcatcaccatcagctgcaccggcaccagcagcgacgtgggcggctacaactacgtgtcctggtatcagcagcaccccggcaaggcccccaagctgatgatctacgaggtgtccaacagacccagcggcgtgagcaacagattcagcggcagcaagagcggcaacaccgccagcctgaccatcagcggcctccaggctgaggacgaggccgactactactgcagcagctacaccagcagctccaccctggtgtttggcggcggaacaaagctgaccgtgctgagagccgacgccgctcccaccgtgtccatcttcccccccagcatggaacagctgacctctggcggagccaccgtggtctgcttcgtgaacaacttctaccccagagacatcagcgtgaagtggaagatcgacggcagcgagcagagggacggcgtgctggacagcgtgaccgaccaggacagcaaggactccacctacagcatgagcagcaccctgagcctgaccaaggtggagtacgagaggcacaacctgtacacctgcgaggtggtgcacaagaccagctccagccccgtggtcaagtccttcaaccggaacgagtgttgagctagcgagctc

SEQ ID NO: 92 - DNA, 13373 bp, Artificial
  VkP-IGKV1-39/J-Ck
ggccggcccacatgaaacaatgggaaccatgtgacaatcacagaggtgttgttactatagcaaaagggattgttactctccacatccctttaagtaacttgaaggcctgatagacccaccctctaagacttcattagacattccctacgaatggttatactctcctgtatactcccaatacaactctaaaatatattattccatatagtccttaggtttgtattaaagtttgacttttttccttcaaaatatctcttgtcacaacagcggctctagagagaaatacattccctccaggcaaatctatgctgcgctggtctgacctgggaccctggggacattgcccctgtgctgagttactaagatgagccagccctgcagctgtgctcagcctgccccatgccctgctgattgatttgcatgttccagagcacagccccctgccctgaagacttttttatgggctggtcgcaccctgtgcaggagtcagtctcagtcaggagccaccatggacatgagagtgcccgcccagctcctggggctcctgctactctggctccgaggtaaggatggagaacactaggaatttactcagccagtgtgctcagtactgactggaacttcagggaagttctctgataacatgattaatagtaagaatatttgtttttatgtttccaatctcaggtgccagatgtgacatccagatgacccagagccccagcagcctgagcgccagcgtgggcgacagagtgaccatcacctgcagagccagccagagcatcagcagctacctgaactggtatcagcagaagcccggcaaggcccccaagctgctgatctacgccgccagctccctgcagagcggcgtgcccagcagattcagcggcagcggctccggcaccgacttcaccctgaccatcagcagcctgcagcccgaggacttcgccacctactactgccagcagagctacagcaccccccccaccttcggccagggcaccaaggtggagatcaaacgtaagtacacttttctcatctttttttatgtgtaagacacaggttttcatgttaggagttaaagtcagttcagaaaatcttgagaaaatggagagggctcattatcagttgacgtggcatacagtgtcagattttctgtttatcaagctagtgagattaggggcaaaaagaggctttagttgagaggaaagtaattaatactatggtcaccatccaagagattggatcggagaataagcatgagtagttattgagatctgggtctgactgcaggtagcgtggtcttctagacgtttaagtgggagatttggaggggatgaggaatgaaggaacttcaggatagaaaagggctgaagtcaagttcagctcctaaaatggatgtgggagcaaactttgaagataaactgaatgacccagaggatgaaacagcgcagatcaaagaggggcctggagctctgagaagagaaggagactcatccgtgttgagtttccacaagtactgtcttgagttttgcaataaaagtgggatagcagagttgagtgagccgtaggctgagttctctcttttgtctcctaagtttttatgactacaaaaatcagtagtatgtcctgaaataatcattaagctgtttgaaagtatgactgcttgccatgtagataccatggcttgctgaataatcagaagaggtgtgactcttattctaaaatttgtcacaaaatgtcaaaatgagagactctgtaggaacgagtccttgacagacagctcaaggggtttttttcctttgtctcatttctacatgaaagtaaatttgaaatgatcttttttattataagagtagaaatacagttgggtttgaactatatgttttaatggccacggttttgtaagacatttggtcctttgttttcccagttattactcgattgtaattttatatcgccagcaatggactgaaacggtccgcaacctcttctttacaactgggtgacctcgcggctgtgccagccatttggcgttcaccctgccgctaagggccatgtgaacccccgcggtagcatcccttgctccgcgtggaccactttcctgaggcacagtgataggaacagagccactaatctgaagagaacagagatgtgacagactacactaatgtgagaaaaacaaggaaagggtgacttattggagatttcagaaataaaatgcatttattattatattcccttattttaattttctattagggaattagaaagggcataaactgctttatccagtgttatattaaaagcttaatgtatataatcttttagaggtaaaatctacagccagcaaaagtcatggtaaatattctttgactgaactctcactaaactcctctaaattatatgtcatattaactggttaaattaatataaatttgtgacatgaccttaactggttaggtaggatatttttcttcatgcaaaaatatgactaataataatttagcacaaaaatatttcccaatactttaattctgtgatagaaaaatgtttaactcagctactataatcccataattttgaaaactatttattagcttttgtgtttgacccttccctagccaaaggcaactatttaaggaccctttaaaactcttgaaactactttagagtcattaagttatttaaccacttttaattactttaaaatgatgtcaattcccttttaactattaatttattttaaggggggaaaggctgctcataattctattgtttttcttggtaaagaactctcagttttcgtttttactacctctgtcacccaagagttggcatctcaacagaggggactttccgagaggccatctggcagttgcttaagatcagaagtgaagtctgccagttcctcccaggcaggtggcccagattacagttgacctgttctggtgtggctaaaaattgtcccatgtggttacaaaccattagaccagggtctgatgaattgctcagaatatttctggacacccaaatacagaccctggcttaaggccctgtccatacagtaggtttagcttggctacaccaaaggaagccatacagaggctaatatcagagtattcttggaagagacaggagaaaatgaaagccagtttctgctcttaccttatgtgcttgtgttcagactcccaaacatcaggagtgtcagataaactggtctgaatctctgtctgaagcatggaactgaaaagaatgtagtttcagggaagaaaggcaatagaaggaagcctgagaatatcttcaaagggtcagactcaatttactttctaaagaagtagctaggaactagggaataacttagaaacaacaagattgtatatatgtgcatcctggccccattgttccttatctgtagggataagcgtgcttttttgtgtgtctgtatataacataactgtttacacataatacactgaaatggagcccttccttgttacttcataccatcctctgtgcttccttcctcaggggccgacgccgctcccaccgtgtccatcttcccccccagcatggaacagctgacctctggcggagccaccgtggtctgcttcgtgaacaacttctaccccagagacatcagcgtgaagtggaagatcgacggcagcgagcagagggacggcgtgctggacagcgtgaccgaccaggacagcaaggactccacctacagcatgagcagcaccctgagcctgaccaaggtggagtacgagaggcacaacctgtacacctgcgaggtggtgcacaagaccagctccagccccgtggtcaagtccttcaaccggaacgagtgttgaagacaaaggtcctgagacgccaccaccagctccccagctccatcctatcttcccttctaaggtcttggaggcttccccacaagcgacctaccactgttgcggtgctccaaacctcctccccacctccttctcctcctcctccctttccttggcttttatcatgctaatatttgcagaaaatattcaataaagtgagtctttgcacttgagatctctgtctttcttactaaatggtagtaatcagttgtttttccagttacctgggtttctcttctaaagaagttaaatgtttagttgccctgaaatccaccacacttaaaggataaataaaaccctccacttgccctggttggctgtccactacatggcagtcctttctaaggttcacgagtactattcatggcttatttctctgggccatggtaggtttgaggaggcatacttcctagttttcttcccctaagtcgtcaaagtcctgaagggggacagtctttacaagcacatgttctgtaatctgattcaacctacccagtaaacttggcgaagcaaagtagaatcattatcacaggaagcaaaggcaacctaaatgtgcaagcaataggaaaatgtggaagcccatcatagtacttggacttcatctgcttttgtgccttcactaagtttttaaacatgagctggctcctatctgccattggcaaggctgggcactacccacaacctacttcaaggacctctataccgtgagattacacacatacatcaaaatttgggaaaagttctaccaagctgagagctgatcaccccactcttaggtgcttatctctgtacaccagaaaccttaagaagcaaccagtattgagagactcatttatgaaagtctaaaactggatacaaccaaaatgtccaccaacagttaaattatgacatgttcacaattgagctattacttaataaggagaattaataaaataaaacttaagagcatagtttaatctcataaacaagataataagcaaaacaaaacattttttcatccatgtaagtttaaaagcaggtaaaatttaaaattaagagagacataagttttgaggtagcaagatggaaactctggggcttggggaatgttctgtctctctgtatgggatgtgaaagttactattgtggaattgggatctatgttcttcctgtatatattgtatacttcataataacttcacctaaagaaatatctaatacccagtgcatacataaaagaggatacaaggaatgaatcatacgtcaaggccagaaagacaataaagtaggggatccaggatcaaatctcccacaaccttgagccttctactattctgccttccagagctcaaagtacaaaacacataattcaaacacatgatccctccttggggtctcttccttcatgcatcgaattagaaatagccatgtataaaatgagatagaagagaccttcatcaacaggtcaaagaatataggtaattttgtctgggtatgaagagcccacgtatcaaaggttacattagggaaggaagaggacactaacagtgactttcattctccccctcttcctggaggcccctgcatttagtccctcgtgggctcatccactcagcacacatttactaagcatcttctcagcctacactctgaaggcagtgcagaataatgttagtgtcccttcccccagttaatatgcagtccagtttccctgctccttccctttctcagtccacataaggatgatgggaaaggacagtcaccaaataggagagggcaaccctttgccttcctacctcttgagaatgtacattattatccactttttgaaacttcttttaattgcttttttttaatttgtcttttcaaatagcataaccttgttcatccatttctgggaaccaaatttatcaatcaacagtgcctctaatctggctattaatacaaaaatgcctcctcaaaatatatatgttcgagtcttatctaaaacagaacccacaataaaaaagaagaaagaatacatataagcatttatataattctgagcaaccttgtgctttgtgaaaaaaatataatctaatgtcacatgctgtattctttttatttaacactggtgaaattataccattagagagaaagaggacagatcactgatcctaggatctagggatgttacagataagaaaacaaatgtgacaaagagctgtcacaaggaggatcttcaaggtcacagaatcactgtcttgatttcagtggtggttacatacatttaaatatgtgataaaatgttgttgaactatattcatatattgtaccaatgtcaaatgcttaattttggctctatagtataattatgcactaaataactatttggacaaagaaaatgatgtttacatcaaaggtgaggccatatttgttaggaacataacttaaaaaccattttggataactaatgaaaagccattttgtgtgccttggcatatcatgcctaagctgtcaccagatagatctaataagacctaagcctcagaagcaagcccctgcccagcaagcaggcagcacagataagagctaaacccaggacaggccatgatatgctaatgaactaccttcaaggtggtgttgctgacctagtgaaccagccccaagctgtgagccccaatagcacaaagctactgcccaaagaaattatacaaaaattggaactttgggaatggtgtgcaggatcgctctgctgtatgcctggaacacagcttctctatgttttgtattgataccagtctagaagcttccaaaactttctcactgaagaagattccccatgtgggacccctacagactcttttgcccaaacaactgcttccctcctggtgtgatatctgttttgcttttatgttagcataatattataaggaatgtttgtgtgaataaaccaaacatattttaaaagcaaatattgtatgcacatcctaattgctaaaaagtttacagctaatagtcccatgctctccacaatactggatccaaataagtcctaatttcaatgttgggcatctttacagagagaaagacattaaaaatgaagagacatgcagagagtgcaccatgccatcgtggagacagactgaagtgacacaactgttagtcaaagaggattaaggacttccagaagccaccaaaggaaggaggtatgaagtggtttctccctcagagtatccagaggagactaaaccaaccaacacctttttgcttaagacttcttgccttcaggactgtgagaaggtagcttcctattgttctaagccccagtatgtggcattttgttaaggtagagtcaagaaaccaataaaatgcagacagacaaaaggatagctgagttttccaggcccttccttcttatttttggttttgttggtggtggtggtggtggtggtgatggtggtggttttgtttatgttttgtttggggagttttttggggtttttttgggttttgtttttgttgttgttttgggggtttttgttgttgttgttgtttgcttttttgttttttgttttttgtttttttgagacagtgtttctctgtatagccctggctgtcctggagttccttctatctctaatgtctacatctcagaggggatcctctaatttcaaatgagcagtagctctccatttttagctcttatttattcatttatttacttacttacttattgtctgtagatgaaagaattttggagtgggaaagggttcatgagcccccagcaactaatgaggagctacagacaattgatgtttctggggaaaggagactcagtttctttgagagtatagcttctgatgggtcaaccatgttcctgtggctgatgtcacacccaggagtatgcagacaacagaaactggagttaatgagttgttttaaaaataaaaaagggcatgaagcttgggatagaaattaaggataaatacaattaaatacaggaaattctgaaagaattaataaaaacatttctttttttaaaaaaaaatccagaattagctatgcttcttcaaaattgcttctggagaactttacaagttaaataagttatattgtagaaaaggtagagaggagaatagtggaagagagagataaggagacttcaaaaggagtggagggagatagaggaggagaaagcagaagcaatggctgatagacacaggataagagggaacagaaaggagaaagaggaagccaggatgggtatttctttgcctatctgtgacttgcacatggtcttggcaattattgatgagttcaaggcttaattcttcacttgtgccaactcaacagagtctttctttcttataaccaggcccccagtatgctcatgtatgtatcaggtcctcttatctccttatagcaatcctgtttataactgggtaactttgtgaagggaaggaagtgcacactgagatgtgctacaactttttaatacaaaattttgaagagtttgtacaatgtatgtataattaataattaatattatgcactttagattttgatttcaactcaagatactaattctatatatatgggttaaatcaatatattaataagtttaatttcacatgcttatttttattgtggttttcgagacagggtttctctgtatagccctggctgtcctggaacccactttgtagaccaggctggcctcaaactcagaaacctacctgcctctgcctctgcctctgcctctgcctctgcctctgcctctgcctctgcctctgcctctgcctctgcctctgcctctgcctctgcctctgcctctgcctctgcctctgcctctgcctctgcctctgcctctgcctctgcctctgcctctgcctctgcctctgcctctgcctctgcctagtgctggaattaaaggtttgcgccaccacgcccggtgaaatttttaaactttatatatgtctcattctatttctatcagataggactgtgtagactgtgctaaactaataaatgtgccctcaaaagtaatcgcaagttgtattgttgttgttttgctttgctttgctttgctttgctttgctttgctttgctttgctttgctttgctttgctttgctttgctttgctttgctttgctttgctttgctttgctttgcttttttgttttgggtttttttccgggggagggagggtggagaaagaatcttactatgaagctctgactgtcctgggaactcactatatagatcaggcttgattcaactcatagagatctgccttcttctgcctcccaagtgctgggaataaaggcatacacctccatgcccagatagtgatcccaagttttagcaaaagtttctagacttgacattaatcgatggagatagacatgaattacacaaagaactaatgtggagtttacctgaatcatactctatactttatcagagattaaattaacatttaataatccagtgccaggctagaggcaccattcaatggcagtgtttgccatcatgcataggcttagtcttcagtgctgaaaggcattgggggcaatattactcattatacagatgagaaactgggaaagacttgcctcagattctctactgaaaggctgagtttgtggcttctagaaaatcttttactttcaatatttttaatgtataatttttttatttccactgattttattttttatttttaacatttataagaaataaatgcaataaaccaaatacatggacaaaaaaatacaagaatcatatgatcacctcaatggaaggaaaaaaaaagaaagaaaaagtctttgataagattcaacattcattctttttttattagatattttcttcatttacatttcaaatgctatccccaaagccccctataccttcccctgccctgctccccaacccacccactcctgctttctggccctggcattcctctgtactgaggcatatgatcttcaaaaaaccaagggcctctcctctcattggtggccgactattaggccatcttttgctacatatgcaactagagacacagctctgggggttactggttagttcatattgttagtcctcctatagagttgcagacccctttagctccttggatactttctctagttccttcattaggggccctgtgtcccatccaatagatgactgtgagcatccacttctgtatttgccaggcactggcatagcctcacgagaaagagagagctatgtcaggatcctgtcagtaaaatctttctggcatatgcaatagtatctgggtttggtggttgtatatgggatggatccccaagtggagcagtctctgaatggtccttccttccatctcagctccaaactttgtctctataactccttccatgggtattttgttccccattctaagaaggagtgaagaatccacactttggtcttccttcttcttgagtttcatatgttgcatcttggatattctaagtttctgggttaatatccacgtatcagtgagtgcatatcatgcgtgttattttgtgattagtttacctcactcaggatgatatcctccagatgcatccatttgcctaagaatttcattaattcactgtttttaattgctgaatagtactccattgtgtaaatgtaccacattttctgtatccattcctctgttgaggggcatctgggttctttccagcttctggctattataaataaggctgctatgagcatagcggagcatgtgtccttatcaagttggaacatcttctaggtatatgcccaggagaggaattgctggatcttccggtagtaccatcaacatgcattcttaataaaagccctagaacaaggaggactgtaggaaacatattccaacataataaaggttatgtatgacaaactcatgaccaatatcatcctaaatgaatgaaaccattaataagctccattaaaatcagaggactgcccactatccctacttctcatccataatgagattgaagcattagctggagcaataaggcaagagaagggatacaaatgggaaaatattaagtcaaattgttttcaattgaagattatattatcttatacccaatgacctcaaattttgactagaaaaattgtagaaattatcaataatttcagcaaagtgttatgatgcaccacatccttattcttctccccagcttctgcttgcttctctcttcttgctcttcatcctttctgtccttccatctgcctgcactcttgtctcaagactgagtgcagcgtgtaactctcctgtgactgagtatctcacaaaacgttctacctgccaaacctggatgagccctttgtctttctgaagctatgaggctctctacatagactcaagaaggaaatgacagggaggaggtaataatgaagtggggaaggctgacattagcattgctcctgtgtggctccttaatttctcatacttcacactgagatgttattaactgtgactcataggtgaagaagccagagctaaggttctcatatttgagtgttatagaatgagtagagcagtagttctcaaactatgggtcatgactcctttatgggtcaaactaccctttcacacaggttgcatatcagatatcctaattttatatacatatatatatgcatatgtatatatatatatttcacaacagtaggaaaattatttagtaatcattttatagttgtgggtcatggcaacatgaggaactgtattaaagggttgcagcattaggaatgttgagacccactgtaatagagaatgaggcttaaggcagggctataaagcccaatggaccatgtgccttttccaacatttgccacatggtaagctctgtatagactttttaaagaacattggtttgtaattttaaatggataagggtcttcactgtctatcacccatctatataataaatacataagttttgattccaccatggattcaaatgcaaaaatcctcaacctaagacatagcagtgaaacattgatgaccaaataggaaatccatgtagagaccttctatcttctgatggctccacaggcaccatcttgcaacagagttctactttgctaccagtaatgaatacagtgtctcaactcctgccattgaatcttcaggaagcccctgaaatgacttgtactacaccatttcttaaagacagaaaagctaagacttagagggaataaatgtcatgcctgagatcatgcaaccaattaagtccaacttggcctgatcaagaggcacaattcaaaagcaatgttgttccttcactagctcttgtgtatggttgctgattccggaagcaaagtatcagtgaatatccctagtgggaaaagacttggaaatcaaatgtctcatttaacagattaggagatgaaacggtagactctgtgtagttgtacacccctgtgatcccatcgctaggaagactgaggcaggaagtcctcgagctcaaaccagcttaggctacacagagaaactatctaaaaaataattactaactacttaataggagattggatgttaagatctggtcactaagaggcagaattgagattcgaagccagtattttctacctggtatgttttaaattgcagtaaggatctaagtgtagatatataataataagattctattgatctctgcaacaacagagagtgttagatttgtttggaaaaaaatattatcagccaacatcttctaccatttcagtatagcacagagtacccacccatatctccccacccatcccccataccagactggttattgattttcatggtgactggcctgagaagattaaaaaaagtaatgctaccttattgggagtgtcccatggaccaagatagcaactgtcatagctaccgtcacactgctttgatcaagaagaccctttgaggaactgaaaacagaaccttaggcacatctgttgctttcgctcccatcctcctccaacagcctgggtggtgcactccacaccctttcaagtttccaaagcctcatacacctgctccctaccccagcacctggccaaggctgtatccagcactgggatgaaaatgataccccacctccatcttgtttgatattactctatctcaagccccaggttagtccccagtcccaatgcttttgcacagtcaaaactcaacttggaataatcagtatccttgaagagttctgatatggtcactgggcccatataccatgtaagacatgtggaaaagatgtttcatggggcccagacacgttctagaagtacctgagagtggcaaaaaatagttgtgctaaatagtttggccatctttaggctgagagactaggaaatacagcgatggactatatcagcattgcaggatagttgtcagtaaacaccccacaacccataacagaagtattctcttctttctatatcccttttccatccatgtagatggctgtcttcatatttgttctagacggccggcc

SEQ ID NO: 93 - DNA, 12892 bp, Artificial
  VkP-IGKV1-39/J-Ck-delta1
ggccggcccacatgaaacaatgggaaccatgtgacaatcacagaggtgttgttactatagcaaaagggattgttactctccacatccctttaagtaacttgaaggcctgatagacccaccctctaagacttcattagacattccctacgaatggttatactctcctgtatactcccaatacaactctaaaatatattattccatatagtccttaggtttgtattaaagtttgacttttttccttcaaaatatctcttgtcacaacagcggctctagagagaaatacattccctccaggcaaatctatgctgcgctggtctgacctgggaccctggggacattgcccctgtgctgagttactaagatgagccagccctgcagctgtgctcagcctgccccatgccctgctgattgatttgcatgttccagagcacagccccctgccctgaagacttttttatgggctggtcgcaccctgtgcaggagtcagtctcagtcaggagccaccatggacatgagagtgcccgcccagctcctggggctcctgctactctggctccgaggtaaggatggagaacactaggaatttactcagccagtgtgctcagtactgactggaacttcagggaagttctctgataacatgattaatagtaagaatatttgtttttatgtttccaatctcaggtgccagatgtgacatccagatgacccagagccccagcagcctgagcgccagcgtgggcgacagagtgaccatcacctgcagagccagccagagcatcagcagctacctgaactggtatcagcagaagcccggcaaggcccccaagctgctgatctacgccgccagctccctgcagagcggcgtgcccagcagattcagcggcagcggctccggcaccgacttcaccctgaccatcagcagcctgcagcccgaggacttcgccacctactactgccagcagagctacagcaccccccccaccttcggccagggcaccaaggtggagatcaaacgtaagtacacttttctcatctttttttatgtgtaagacacaggttttcatgttaggagttaaagtcagttcagaaaatcttgagaaaatggagagggctcattatcagttgacgtggcatacagtgtcagattttctgtttatcaagctagtgagattaggggcaaaaagaggctttagttgagaggaaagtaattaatactatggtcaccatccaagagattggatcggagaataagcatgagtagttattgagatctgggtctgactgcaggtagcgtggtcttctagacgtttaagtgggagatttggaggggatgaggaatgaaggaacttcaggatagaaaagggctgaagtcaagttcagctcctaaaatggatgtgggagcaaactttgaagataaactgaatgacccagaggatgaaacagcgcagatcaaagaggggcctggagctctgagaagagaaggagactcatccgtgttgagtttccacaagtactgtcttgagttttgcaataaaagtgggatagcagagttgagtgagccgtaggctgagttctctcttttgtctcctaagtttttatgactacaaaaatcagtagtatgtcctgaaataatcattaagctgtttgaaagtatgactgcttgccatgtagataccatggcttgctgaataatcagaagaggtgtgactcttattctaaaatttgtcacaaaatgtcaaaatgagagactctgtaggaacgagtccttgacagacagctcaaggggtttttttcctttgtctcatttctacatgaaagtaaatttgaaatgatcttttttattataagagtagaaatacagttgggtttgaactatatgttttaatggccacggttttgtaagacatttggtcctttgttttcccagttattactcgattgtaattttatatcgccagcaatggactgaaacggtccgcaacctcttctttacaactgggtgacctcgcggctgtgccagccatttggcgttcaccctgccgctaagggccatgtgaacccccgcggtagcatcccttgctccgcgtggaccactttcctgaggcacagtgataggaacagagccactaatctgaagagaacagagatgtgacagactacactaatgtgagaaaaacaaggaaagggtgacttattggagatttcagaaataaaatgcatttattattatattcccttattttaattttctattagggaattagaaagggcataaactgctttatccagtgttatattaaaagcttaatgtatataatcttttagaggtaaaatctacagccagcaaaagtcatggtaaatattctttgactgaactctcactaaactcctctaaattatatgtcatattaactggttaaattaatataaatttgtgacatgaccttaactggttaggtaggatatttttcttcatgcaaaaatatgactaataataatttagcacaaaaatatttcccaatactttaattctgtgatagaaaaatgtttaactcagctactataatcccataattttgaaaactatttatttggctacaccaaaggaagccatacagaggctaatatcagagtattcttggaagagacaggagaaaatgaaagccagtttctgctcttaccttatgtgcttgtgttcagactcccaaacatcaggagtgtcagataaactggtctgaatctctgtctgaagcatggaactgaaaagaatgtagtttcagggaagaaaggcaatagaaggaagcctgagaatatcttcaaagggtcagactcaatttactttctaaagaagtagctaggaactagggaataacttagaaacaacaagattgtatatatgtgcatcctggccccattgttccttatctgtagggataagcgtgcttttttgtgtgtctgtatataacataactgtttacacataatacactgaaatggagcccttccttgttacttcataccatcctctgtgcttccttcctcaggggccgacgccgctcccaccgtgtccatcttcccccccagcatggaacagctgacctctggcggagccaccgtggtctgcttcgtgaacaacttctaccccagagacatcagcgtgaagtggaagatcgacggcagcgagcagagggacggcgtgctggacagcgtgaccgaccaggacagcaaggactccacctacagcatgagcagcaccctgagcctgaccaaggtggagtacgagaggcacaacctgtacacctgcgaggtggtgcacaagaccagctccagccccgtggtcaagtccttcaaccggaacgagtgttgaagacaaaggtcctgagacgccaccaccagctccccagctccatcctatcttcccttctaaggtcttggaggcttccccacaagcgacctaccactgttgcggtgctccaaacctcctccccacctccttctcctcctcctccctttccttggcttttatcatgctaatatttgcagaaaatattcaataaagtgagtctttgcacttgagatctctgtctttcttactaaatggtagtaatcagttgtttttccagttacctgggtttctcttctaaagaagttaaatgtttagttgccctgaaatccaccacacttaaaggataaataaaaccctccacttgccctggttggctgtccactacatggcagtcctttctaaggttcacgagtactattcatggcttatttctctgggccatggtaggtttgaggaggcatacttcctagttttcttcccctaagtcgtcaaagtcctgaagggggacagtctttacaagcacatgttctgtaatctgattcaacctacccagtaaacttggcgaagcaaagtagaatcattatcacaggaagcaaaggcaacctaaatgtgcaagcaataggaaaatgtggaagcccatcatagtacttggacttcatctgcttttgtgccttcactaagtttttaaacatgagctggctcctatctgccattggcaaggctgggcactacccacaacctacttcaaggacctctataccgtgagattacacacatacatcaaaatttgggaaaagttctaccaagctgagagctgatcaccccactcttaggtgcttatctctgtacaccagaaaccttaagaagcaaccagtattgagagactcatttatgaaagtctaaaactggatacaaccaaaatgtccaccaacagttaaattatgacatgttcacaattgagctattacttaataaggagaattaataaaataaaacttaagagcatagtttaatctcataaacaagataataagcaaaacaaaacattttttcatccatgtaagtttaaaagcaggtaaaatttaaaattaagagagacataagttttgaggtagcaagatggaaactctggggcttggggaatgttctgtctctctgtatgggatgtgaaagttactattgtggaattgggatctatgttcttcctgtatatattgtatacttcataataacttcacctaaagaaatatctaatacccagtgcatacataaaagaggatacaaggaatgaatcatacgtcaaggccagaaagacaataaagtaggggatccaggatcaaatctcccacaaccttgagccttctactattctgccttccagagctcaaagtacaaaacacataattcaaacacatgatccctccttggggtctcttccttcatgcatcgaattagaaatagccatgtataaaatgagatagaagagaccttcatcaacaggtcaaagaatataggtaattttgtctgggtatgaagagcccacgtatcaaaggttacattagggaaggaagaggacactaacagtgactttcattctccccctcttcctggaggcccctgcatttagtccctcgtgggctcatccactcagcacacatttactaagcatcttctcagcctacactctgaaggcagtgcagaataatgttagtgtcccttcccccagttaatatgcagtccagtttccctgctccttccctttctcagtccacataaggatgatgggaaaggacagtcaccaaataggagagggcaaccctttgccttcctacctcttgagaatgtacattattatccactttttgaaacttcttttaattgcttttttttaatttgtcttttcaaatagcataaccttgttcatccatttctgggaaccaaatttatcaatcaacagtgcctctaatctggctattaatacaaaaatgcctcctcaaaatatatatgttcgagtcttatctaaaacagaacccacaataaaaaagaagaaagaatacatataagcatttatataattctgagcaaccttgtgctttgtgaaaaaaatataatctaatgtcacatgctgtattctttttatttaacactggtgaaattataccattagagagaaagaggacagatcactgatcctaggatctagggatgttacagataagaaaacaaatgtgacaaagagctgtcacaaggaggatcttcaaggtcacagaatcactgtcttgatttcagtggtggttacatacatttaaatatgtgataaaatgttgttgaactatattcatatattgtaccaatgtcaaatgcttaattttggctctatagtataattatgcactaaataactatttggacaaagaaaatgatgtttacatcaaaggtgaggccatatttgttaggaacataacttaaaaaccattttggataactaatgaaaagccattttgtgtgccttggcatatcatgcctaagctgtcaccagatagatctaataagacctaagcctcagaagcaagcccctgcccagcaagcaggcagcacagataagagctaaacccaggacaggccatgatatgctaatgaactaccttcaaggtggtgttgctgacctagtgaaccagccccaagctgtgagccccaatagcacaaagctactgcccaaagaaattatacaaaaattggaactttgggaatggtgtgcaggatcgctctgctgtatgcctggaacacagcttctctatgttttgtattgataccagtctagaagcttccaaaactttctcactgaagaagattccccatgtgggacccctacagactcttttgcccaaacaactgcttccctcctggtgtgatatctgttttgcttttatgttagcataatattataaggaatgtttgtgtgaataaaccaaacatattttaaaagcaaatattgtatgcacatcctaattgctaaaaagtttacagctaatagtcccatgctctccacaatactggatccaaataagtcctaatttcaatgttgggcatctttacagagagaaagacattaaaaatgaagagacatgcagagagtgcaccatgccatcgtggagacagactgaagtgacacaactgttagtcaaagaggattaaggacttccagaagccaccaaaggaaggaggtatgaagtggtttctccctcagagtatccagaggagactaaaccaaccaacacctttttgcttaagacttcttgccttcaggactgtgagaaggtagcttcctattgttctaagccccagtatgtggcattttgttaaggtagagtcaagaaaccaataaaatgcagacagacaaaaggatagctgagttttccaggcccttccttcttatttttggttttgttggtggtggtggtggtggtggtgatggtggtggttttgtttatgttttgtttggggagttttttggggtttttttgggttttgtttttgttgttgttttgggggtttttgttgttgttgttgtttgcttttttgttttttgttttttgtttttttgagacagtgtttctctgtatagccctggctgtcctggagttccttctatctctaatgtctacatctcagaggggatcctctaatttcaaatgagcagtagctctccatttttagctcttatttattcatttatttacttacttacttattgtctgtagatgaaagaattttggagtgggaaagggttcatgagcccccagcaactaatgaggagctacagacaattgatgtttctggggaaaggagactcagtttctttgagagtatagcttctgatgggtcaaccatgttcctgtggctgatgtcacacccaggagtatgcagacaacagaaactggagttaatgagttgttttaaaaataaaaaagggcatgaagcttgggatagaaattaaggataaatacaattaaatacaggaaattctgaaagaattaataaaaacatttctttttttaaaaaaaaatccagaattagctatgcttcttcaaaattgcttctggagaactttacaagttaaataagttatattgtagaaaaggtagagaggagaatagtggaagagagagataaggagacttcaaaaggagtggagggagatagaggaggagaaagcagaagcaatggctgatagacacaggataagagggaacagaaaggagaaagaggaagccaggatgggtatttctttgcctatctgtgacttgcacatggtcttggcaattattgatgagttcaaggcttaattcttcacttgtgccaactcaacagagtctttctttcttataaccaggcccccagtatgctcatgtatgtatcaggtcctcttatctccttatagcaatcctgtttataactgggtaactttgtgaagggaaggaagtgcacactgagatgtgctacaactttttaatacaaaattttgaagagtttgtacaatgtatgtataattaataattaatattatgcactttagattttgatttcaactcaagatactaattctatatatatgggttaaatcaatatattaataagtttaatttcacatgcttatttttattgtggttttcgagacagggtttctctgtatagccctggctgtcctggaacccactttgtagaccaggctggcctcaaactcagaaacctacctgcctctgcctctgcctctgcctctgcctctgcctctgcctctgcctctgcctctgcctctgcctctgcctctgcctctgcctctgcctctgcctctgcctctgcctctgcctctgcctctgcctctgcctctgcctctgcctctgcctctgcctctgcctctgcctctgcctctgcctagtgctggaattaaaggtttgcgccaccacgcccggtgaaatttttaaactttatatatgtctcattctatttctatcagataggactgtgtagactgtgctaaactaataaatgtgccctcaaaagtaatcgcaagttgtattgttgttgttttgctttgctttgctttgctttgctttgctttgctttgctttgctttgctttgctttgctttgctttgctttgctttgctttgctttgctttgctttgctttgcttttttgttttgggtttttttccgggggagggagggtggagaaagaatcttactatgaagctctgactgtcctgggaactcactatatagatcaggcttgattcaactcatagagatctgccttcttctgcctcccaagtgctgggaataaaggcatacacctccatgcccagatagtgatcccaagttttagcaaaagtttctagacttgacattaatcgatggagatagacatgaattacacaaagaactaatgtggagtttacctgaatcatactctatactttatcagagattaaattaacatttaataatccagtgccaggctagaggcaccattcaatggcagtgtttgccatcatgcataggcttagtcttcagtgctgaaaggcattgggggcaatattactcattatacagatgagaaactgggaaagacttgcctcagattctctactgaaaggctgagtttgtggcttctagaaaatcttttactttcaatatttttaatgtataatttttttatttccactgattttattttttatttttaacatttataagaaataaatgcaataaaccaaatacatggacaaaaaaatacaagaatcatatgatcacctcaatggaaggaaaaaaaaagaaagaaaaagtctttgataagattcaacattcattctttttttattagatattttcttcatttacatttcaaatgctatccccaaagccccctataccttcccctgccctgctccccaacccacccactcctgctttctggccctggcattcctctgtactgaggcatatgatcttcaaaaaaccaagggcctctcctctcattggtggccgactattaggccatcttttgctacatatgcaactagagacacagctctgggggttactggttagttcatattgttagtcctcctatagagttgcagacccctttagctccttggatactttctctagttccttcattaggggccctgtgtcccatccaatagatgactgtgagcatccacttctgtatttgccaggcactggcatagcctcacgagaaagagagagctatgtcaggatcctgtcagtaaaatctttctggcatatgcaatagtatctgggtttggtggttgtatatgggatggatccccaagtggagcagtctctgaatggtccttccttccatctcagctccaaactttgtctctataactccttccatgggtattttgttccccattctaagaaggagtgaagaatccacactttggtcttccttcttcttgagtttcatatgttgcatcttggatattctaagtttctgggttaatatccacgtatcagtgagtgcatatcatgcgtgttattttgtgattagtttacctcactcaggatgatatcctccagatgcatccatttgcctaagaatttcattaattcactgtttttaattgctgaatagtactccattgtgtaaatgtaccacattttctgtatccattcctctgttgaggggcatctgggttctttccagcttctggctattataaataaggctgctatgagcatagcggagcatgtgtccttatcaagttggaacatcttctaggtatatgcccaggagaggaattgctggatcttccggtagtaccatcaacatgcattcttaataaaagccctagaacaaggaggactgtaggaaacatattccaacataataaaggttatgtatgacaaactcatgaccaatatcatcctaaatgaatgaaaccattaataagctccattaaaatcagaggactgcccactatccctacttctcatccataatgagattgaagcattagctggagcaataaggcaagagaagggatacaaatgggaaaatattaagtcaaattgttttcaattgaagattatattatcttatacccaatgacctcaaattttgactagaaaaattgtagaaattatcaataatttcagcaaagtgttatgatgcaccacatccttattcttctccccagcttctgcttgcttctctcttcttgctcttcatcctttctgtccttccatctgcctgcactcttgtctcaagactgagtgcagcgtgtaactctcctgtgactgagtatctcacaaaacgttctacctgccaaacctggatgagccctttgtctttctgaagctatgaggctctctacatagactcaagaaggaaatgacagggaggaggtaataatgaagtggggaaggctgacattagcattgctcctgtgtggctccttaatttctcatacttcacactgagatgttattaactgtgactcataggtgaagaagccagagctaaggttctcatatttgagtgttatagaatgagtagagcagtagttctcaaactatgggtcatgactcctttatgggtcaaactaccctttcacacaggttgcatatcagatatcctaattttatatacatatatatatgcatatgtatatatatatatttcacaacagtaggaaaattatttagtaatcattttatagttgtgggtcatggcaacatgaggaactgtattaaagggttgcagcattaggaatgttgagacccactgtaatagagaatgaggcttaaggcagggctataaagcccaatggaccatgtgccttttccaacatttgccacatggtaagctctgtatagactttttaaagaacattggtttgtaattttaaatggataagggtcttcactgtctatcacccatctatataataaatacataagttttgattccaccatggattcaaatgcaaaaatcctcaacctaagacatagcagtgaaacattgatgaccaaataggaaatccatgtagagaccttctatcttctgatggctccacaggcaccatcttgcaacagagttctactttgctaccagtaatgaatacagtgtctcaactcctgccattgaatcttcaggaagcccctgaaatgacttgtactacaccatttcttaaagacagaaaagctaagacttagagggaataaatgtcatgcctgagatcatgcaaccaattaagtccaacttggcctgatcaagaggcacaattcaaaagcaatgttgttccttcactagctcttgtgtatggttgctgattccggaagcaaagtatcagtgaatatccctagtgggaaaagacttggaaatcaaatgtctcatttaacagattaggagatgaaacggtagactctgtgtagttgtacacccctgtgatcccatcgctaggaagactgaggcaggaagtcctcgagctcaaaccagcttaggctacacagagaaactatctaaaaaataattactaactacttaataggagattggatgttaagatctggtcactaagaggcagaattgagattcgaagccagtattttctacctggtatgttttaaattgcagtaaggatctaagtgtagatatataataataagattctattgatctctgcaacaacagagagtgttagatttgtttggaaaaaaatattatcagccaacatcttctaccatttcagtatagcacagagtacccacccatatctccccacccatcccccataccagactggttattgattttcatggtgactggcctgagaagattaaaaaaagtaatgctaccttattgggagtgtcccatggaccaagatagcaactgtcatagctaccgtcacactgctttgatcaagaagaccctttgaggaactgaaaacagaaccttaggcacatctgttgctttcgctcccatcctcctccaacagcctgggtggtgcactccacaccctttcaagtttccaaagcctcatacacctgctccctaccccagcacctggccaaggctgtatccagcactgggatgaaaatgataccccacctccatcttgtttgatattactctatctcaagccccaggttagtccccagtcccaatgcttttgcacagtcaaaactcaacttggaataatcagtatccttgaagagttctgatatggtcactgggcccatataccatgtaagacatgtggaaaagatgtttcatggggcccagacacgttctagaagtacctgagagtggcaaaaaatagttgtgctaaatagtttggccatctttaggctgagagactaggaaatacagcgatggactatatcagcattgcaggatagttgtcagtaaacaccccacaacccataacagaagtattctcttctttctatatcccttttccatccatgtagatggctgtcttcatatttgttctagacggccggcc

SEQ ID NO: 94 - DNA, 6425 bp, VkP-IGKV1-39/J-Ck-delta2
ggccggcccacatgaaacaatgggaaccatgtgacaatcacagaggtgttgttactatagcaaaagggattgttactctccacatccctttaagtaacttgaaggcctgatagacccaccctctaagacttcattagacattccctacgaatggttatactctcctgtatactcccaatacaactctaaaatatattattccatatagtccttaggtttgtattaaagtttgacttttttccttcaaaatatctcttgtcacaacagcggctctagagagaaatacattccctccaggcaaatctatgctgcgctggtctgacctgggaccctggggacattgcccctgtgctgagttactaagatgagccagccctgcagctgtgctcagcctgccccatgccctgctgattgatttgcatgttccagagcacagccccctgccctgaagacttttttatgggctggtcgcaccctgtgcaggagtcagtctcagtcaggagccaccatggacatgagagtgcccgcccagctcctggggctcctgctactctggctccgaggtaaggatggagaacactaggaatttactcagccagtgtgctcagtactgactggaacttcagggaagttctctgataacatgattaatagtaagaatatttgtttttatgtttccaatctcaggtgccagatgtgacatccagatgacccagagccccagcagcctgagcgccagcgtgggcgacagagtgaccatcacctgcagagccagccagagcatcagcagctacctgaactggtatcagcagaagcccggcaaggcccccaagctgctgatctacgccgccagctccctgcagagcggcgtgcccagcagattcagcggcagcggctccggcaccgacttcaccctgaccatcagcagcctgcagcccgaggacttcgccacctactactgccagcagagctacagcaccccccccaccttcggccagggcaccaaggtggagatcaaacgtaagtacacttttctcatctttttttatgtgtaagacacaggttttcatgttaggagttaaagtcagttcagaaaatcttgagaaaatggagagggctcattatcagttgacgtggcatacagtgtcagattttctgtttatcaagctagtgagattaggggcaaaaagaggctttagttgagaggaaagtaattaatactatggtcaccatccaagagattggatcggagaataagcatgagtagttattgagatctgggtctgactgcaggtagcgtggtcttctagacgtttaagtgggagatttggaggggatgaggaatgaaggaacttcaggatagaaaagggctgaagtcaagttcagctcctaaaatggatgtgggagcaaactttgaagataaactgaatgacccagaggatgaaacagcgcagatcaaagaggggcctggagctctgagaagagaaggagactcatccgtgttgagtttccacaagtactgtcttgagttttgcaataaaagtgggatagcagagttgagtgagccgtaggctgagttctctcttttgtctcctaagtttttatgactacaaaaatcagtagtatgtcctgaaataatcattaagctgtttgaaagtatgactgcttgccatgtagataccatggcttgctgaataatcagaagaggtgtgactcttattctaaaatttgtcacaaaatgtcaaaatgagagactctgtaggaacgagtccttgacagacagctcaaggggtttttttcctttgtctcatttctacatgaaagtaaatttgaaatgatcttttttattataagagtagaaatacagttgggtttgaactatatgttttaatggccacggttttgtaagacatttggtcctttgttttcccagttattactcgattgtaattttatatcgccagcaatggactgaaacggtccgcaacctcttctttacaactgggtgacctcgcggctgtgccagccatttggcgttcaccctgccgctaagggccatgtgaacccccgcggtagcatcccttgctccgcgtggaccactttcctgaggcacagtgataggaacagagccactaatctgaagagaacagagatgtgacagactacactaatgtgagaaaaacaaggaaagggtgacttattggagatttcagaaataaaatgcatttattattatattcccttattttaattttctattagggaattagaaagggcataaactgctttatccagtgttatattaaaagcttaatgtatataatcttttagaggtaaaatctacagccagcaaaagtcatggtaaatattctttgactgaactctcactaaactcctctaaattatatgtcatattaactggttaaattaatataaatttgtgacatgaccttaactggttaggtaggatatttttcttcatgcaaaaatatgactaataataatttagcacaaaaatatttcccaatactttaattctgtgatagaaaaatgtttaactcagctactataatcccataattttgaaaactatttatttggctacaccaaaggaagccatacagaggctaatatcagagtattcttggaagagacaggagaaaatgaaagccagtttctgctcttaccttatgtgcttgtgttcagactcccaaacatcaggagtgtcagataaactggtctgaatctctgtctgaagcatggaactgaaaagaatgtagtttcagggaagaaaggcaatagaaggaagcctgagaatatcttcaaagggtcagactcaatttactttctaaagaagtagctaggaactagggaataacttagaaacaacaagattgtatatatgtgcatcctggccccattgttccttatctgtagggataagcgtgcttttttgtgtgtctgtatataacataactgtttacacataatacactgaaatggagcccttccttgttacttcataccatcctctgtgcttccttcctcaggggccgacgccgctcccaccgtgtccatcttcccccccagcatggaacagctgacctctggcggagccaccgtggtctgcttcgtgaacaacttctaccccagagacatcagcgtgaagtggaagatcgacggcagcgagcagagggacggcgtgctggacagcgtgaccgaccaggacagcaaggactccacctacagcatgagcagcaccctgagcctgaccaaggtggagtacgagaggcacaacctgtacacctgcgaggtggtgcacaagaccagctccagccccgtggtcaagtccttcaaccggaacgagtgttgaagacaaaggtcctgagacgccaccaccagctccccagctccatcctatcttcccttctaaggtcttggaggcttccccacaagcgacctaccactgttgcggtgctccaaacctcctccccacctccttctcctcctcctccctttccttggcttttatcatgctaatatttgcagaaaatattcaataaagtgagtctttgcacttgagatctctgtctttcttactaaatggtagtaatcagttgtttttccagttacctgggtttctcttctaaagaagttaaatgtttagttgccctgaaatccaccacacttaaaggataaataaaaccctccacttgccctggttggctgtccactacatggcagtcctttctaaggttcacgagtactattcatggcttatttctctgggccatggtaggtttgaggaggcatacttcctagttttcttcccctaagtcgtcaaagtcctgaagggggacagtctttacaagcacatgttctgtaatctgattcaacctacccagtaaacttggcgaagcaaagtagaatcattatcacaggaagcaaaggcaacctaaatgtgcaagcaataggaaaatgtggaagcccatcatagtacttggacttcatctgcttttgtgccttcactaagtttttaaacatgagctggctcctatctgccattggcaaggctgggcactacccacaacctacttcaaggacctctataccgtgagattacacacatacatcaaaatttgggaaaagttctaccaagctgagagctgatcaccccactcttaggtgcttatctctgtacaccagaaaccttaagaagcaaccagtattgagagactcatttatgaaagtctaaaactggatacaaccaaaatgtccaccaacagttaaattatgacatgttcacaattgagctattacttaataaggagaattaataaaataaaacttaagagcatagtttaatctcataaacaagataataagcaaaacaaaacattttttcatccatgtaagtttaaaagcaggtaaaatttaaaattaagagagacataagttttgaggtagcaagatggaaactctggggcttggggaatgttctgtctctctgtatgggatgtgaaagttactattgtggaattgggatctatgttcttcctgtatatattgtatacttcataataacttcacctaaagaaatatctaatacccagtgcatacataaaagaggatacaaggaatgaatcatacgtcaaggccagaaagacaataaagtaggggatccaggatcaaatctcccacaaccttgagccttctactattctgccttccagagctcaaagtacaaaacacataattcaaacacatgatccctccttggggtctcttccttcatgcatcgaattagaaatagccatgtataaaatgagatagaagagaccttcatcaacaggtcaaagaatataggtaattttgtctgggtatgaagagcccacgtatcaaaggttacattagggaaggaagaggacactaacagtgactttcattctccccctcttcctggaggcccctgcatttagtccctcgtgggctcatccactcagcacacatttactaagcatcttctcagcctacactctgaaggcagtgcagaataatgttagtgtcccttcccccagttaatatgcagtccagtttccctgctccttccctttctcagtccacataaggatgatgggaaaggacagtcaccaaataggagagggcaaccctttgccttcctacctcttgagaatgtacattattatccactttttgaaacttcttttaattgcttttttttaatttgtcttttcaaatagcataaccttgttcatccatttctgggaaccaaatttatcaatcaacagtgcctctaatctggctattaatacaaaaatgcctcctcaaaatatatatgttcgagtcttatctaaaacagaacccacaataaaaaagaagaaagaatacatataagcatttatataattctgagcaaccttgtgctttgtgaaaaaaatataatctaatgtcacatgctgtattctttttatttaacactggtgaaattataccattagagagaaagaggacagatcactgatcctaggatctagggatgttacagataagaaaacaaatgtgacaaagagctgtcacaaggaggatcttcaaggtcacagaatcactgtcttgatttcagtggtggttacatacatttaaatatgtgataaaatgttgttgaactatattcatatattgtaccaatgtcaaatgcttaattttggctctatagtataattatgcactaaataactatttggacaaagaaaatgatgtttacatcaaaggtgaggccatatttgttaggaacataacttaaaaaccattttggataactaatgaaaagccattttgtgtgccttggcatatcatgcctaagctgtcaccagatagatctaataagacctaagcctcagaagcaagcccctgcccagcaagcaggcagcacagataagagctaaacccaggacaggccatgatatgctaatgaactaccttcaaggtggtgttgctgacctagtgaaccagccccaagctgtgagccccaatagcacaaagctactgcccaaagaaattatacaaaaattggaactttgggaatggtgtgcaggatcgctctgctgtatgcctggaacacagcttctctatgttttgtattgataccagtctagaagcttccaaaactttctcactgaagaagattccccatgtgggacccctacagactcttttgcccaaacaactgcttccctcctggtgtgatcatggaccaagatagcaactgtcatagctaccgtcacactgctttgatcaagaagaccctttgaggaactgaaaacagaaccttaggcacatctgttgctttcgctcccatcctcctccaacagcatggctgtcttcatatttgttctagacggccggcc

SEQ ID NO: 95 - DNA, 13382 bp, Artificial
  VkP-IGLV2-14/J-Ck
ggccggcccacatgaaacaatgggaaccatgtgacaatcacagaggtgttgttactatagcaaaagggattgttactctccacatccctttaagtaacttgaaggcctgatagacccaccctctaagacttcattagacattccctacgaatggttatactctcctgtatactcccaatacaactctaaaatatattattccatatagtccttaggtttgtattaaagtttgacttttttccttcaaaatatctcttgtcacaacagcggctctagagagaaatacattccctccaggcaaatctatgctgcgctggtctgacctgggaccctggggacattgcccctgtgctgagttactaagatgagccagccctgcagctgtgctcagcctgccccatgccctgctgattgatttgcatgttccagagcacagccccctgccctgaagacttttttatgggctggtcgcaccctgtgcaggagtcagtctcagtcaggagccaccatggacatgagagtgcccgcccagctcctggggctcctgctactctggctccgaggtaaggatggagaacactaggaatttactcagccagtgtgctcagtactgactggaacttcagggaagttctctgataacatgattaatagtaagaatatttgtttttatgtttccaatctcaggtgccagatgtcagtctgccctgacccagcccgcctctgtgtctggcagccctggccagagcatcaccatcagctgcaccggcaccagcagcgacgtgggcggctacaactacgtgtcctggtatcagcagcaccccggcaaggcccccaagctgatgatctacgaggtgtccaacagacccagcggcgtgagcaacagattcagcggcagcaagagcggcaacaccgccagcctgaccatcagcggcctccaggctgaggacgaggccgactactactgcagcagctacaccagcagctccaccctggtgtttggcggcggaacaaagctgaccgtgctgcgtaagtacacttttctcatctttttttatgtgtaagacacaggttttcatgttaggagttaaagtcagttcagaaaatcttgagaaaatggagagggctcattatcagttgacgtggcatacagtgtcagattttctgtttatcaagctagtgagattaggggcaaaaagaggctttagttgagaggaaagtaattaatactatggtcaccatccaagagattggatcggagaataagcatgagtagttattgagatctgggtctgactgcaggtagcgtggtcttctagacgtttaagtgggagatttggaggggatgaggaatgaaggaacttcaggatagaaaagggctgaagtcaagttcagctcctaaaatggatgtgggagcaaactttgaagataaactgaatgacccagaggatgaaacagcgcagatcaaagaggggcctggagctctgagaagagaaggagactcatccgtgttgagtttccacaagtactgtcttgagttttgcaataaaagtgggatagcagagttgagtgagccgtaggctgagttctctcttttgtctcctaagtttttatgactacaaaaatcagtagtatgtcctgaaataatcattaagctgtttgaaagtatgactgcttgccatgtagataccatggcttgctgaataatcagaagaggtgtgactcttattctaaaatttgtcacaaaatgtcaaaatgagagactctgtaggaacgagtccttgacagacagctcaaggggtttttttcctttgtctcatttctacatgaaagtaaatttgaaatgatcttttttattataagagtagaaatacagttgggtttgaactatatgttttaatggccacggttttgtaagacatttggtcctttgttttcccagttattactcgattgtaattttatatcgccagcaatggactgaaacggtccgcaacctcttctttacaactgggtgacctcgcggctgtgccagccatttggcgttcaccctgccgctaagggccatgtgaacccccgcggtagcatcccttgctccgcgtggaccactttcctgaggcacagtgataggaacagagccactaatctgaagagaacagagatgtgacagactacactaatgtgagaaaaacaaggaaagggtgacttattggagatttcagaaataaaatgcatttattattatattcccttattttaattttctattagggaattagaaagggcataaactgctttatccagtgttatattaaaagcttaatgtatataatcttttagaggtaaaatctacagccagcaaaagtcatggtaaatattctttgactgaactctcactaaactcctctaaattatatgtcatattaactggttaaattaatataaatttgtgacatgaccttaactggttaggtaggatatttttcttcatgcaaaaatatgactaataataatttagcacaaaaatatttcccaatactttaattctgtgatagaaaaatgtttaactcagctactataatcccataattttgaaaactatttattagcttttgtgtttgacccttccctagccaaaggcaactatttaaggaccctttaaaactcttgaaactactttagagtcattaagttatttaaccacttttaattactttaaaatgatgtcaattcccttttaactattaatttattttaaggggggaaaggctgctcataattctattgtttttcttggtaaagaactctcagttttcgtttttactacctctgtcacccaagagttggcatctcaacagaggggactttccgagaggccatctggcagttgcttaagatcagaagtgaagtctgccagttcctcccaggcaggtggcccagattacagttgacctgttctggtgtggctaaaaattgtcccatgtggttacaaaccattagaccagggtctgatgaattgctcagaatatttctggacacccaaatacagaccctggcttaaggccctgtccatacagtaggtttagcttggctacaccaaaggaagccatacagaggctaatatcagagtattcttggaagagacaggagaaaatgaaagccagtttctgctcttaccttatgtgcttgtgttcagactcccaaacatcaggagtgtcagataaactggtctgaatctctgtctgaagcatggaactgaaaagaatgtagtttcagggaagaaaggcaatagaaggaagcctgagaatatcttcaaagggtcagactcaatttactttctaaagaagtagctaggaactagggaataacttagaaacaacaagattgtatatatgtgcatcctggccccattgttccttatctgtagggataagcgtgcttttttgtgtgtctgtatataacataactgtttacacataatacactgaaatggagcccttccttgttacttcataccatcctctgtgcttccttcctcaggggccgacgccgctcccaccgtgtccatcttcccccccagcatggaacagctgacctctggcggagccaccgtggtctgcttcgtgaacaacttctaccccagagacatcagcgtgaagtggaagatcgacggcagcgagcagagggacggcgtgctggacagcgtgaccgaccaggacagcaaggactccacctacagcatgagcagcaccctgagcctgaccaaggtggagtacgagaggcacaacctgtacacctgcgaggtggtgcacaagaccagctccagccccgtggtcaagtccttcaaccggaacgagtgttgaagacaaaggtcctgagacgccaccaccagctccccagctccatcctatcttcccttctaaggtcttggaggcttccccacaagcgacctaccactgttgcggtgctccaaacctcctccccacctccttctcctcctcctccctttccttggcttttatcatgctaatatttgcagaaaatattcaataaagtgagtctttgcacttgagatctctgtctttcttactaaatggtagtaatcagttgtttttccagttacctgggtttctcttctaaagaagttaaatgtttagttgccctgaaatccaccacacttaaaggataaataaaaccctccacttgccctggttggctgtccactacatggcagtcctttctaaggttcacgagtactattcatggcttatttctctgggccatggtaggtttgaggaggcatacttcctagttttcttcccctaagtcgtcaaagtcctgaagggggacagtctttacaagcacatgttctgtaatctgattcaacctacccagtaaacttggcgaagcaaagtagaatcattatcacaggaagcaaaggcaacctaaatgtgcaagcaataggaaaatgtggaagcccatcatagtacttggacttcatctgcttttgtgccttcactaagtttttaaacatgagctggctcctatctgccattggcaaggctgggcactacccacaacctacttcaaggacctctataccgtgagattacacacatacatcaaaatttgggaaaagttctaccaagctgagagctgatcaccccactcttaggtgcttatctctgtacaccagaaaccttaagaagcaaccagtattgagagactcatttatgaaagtctaaaactggatacaaccaaaatgtccaccaacagttaaattatgacatgttcacaattgagctattacttaataaggagaattaataaaataaaacttaagagcatagtttaatctcataaacaagataataagcaaaacaaaacattttttcatccatgtaagtttaaaagcaggtaaaatttaaaattaagagagacataagttttgaggtagcaagatggaaactctggggcttggggaatgttctgtctctctgtatgggatgtgaaagttactattgtggaattgggatctatgttcttcctgtatatattgtatacttcataataacttcacctaaagaaatatctaatacccagtgcatacataaaagaggatacaaggaatgaatcatacgtcaaggccagaaagacaataaagtaggggatccaggatcaaatctcccacaaccttgagccttctactattctgccttccagagctcaaagtacaaaacacataattcaaacacatgatccctccttggggtctcttccttcatgcatcgaattagaaatagccatgtataaaatgagatagaagagaccttcatcaacaggtcaaagaatataggtaattttgtctgggtatgaagagcccacgtatcaaaggttacattagggaaggaagaggacactaacagtgactttcattctccccctcttcctggaggcccctgcatttagtccctcgtgggctcatccactcagcacacatttactaagcatcttctcagcctacactctgaaggcagtgcagaataatgttagtgtcccttcccccagttaatatgcagtccagtttccctgctccttccctttctcagtccacataaggatgatgggaaaggacagtcaccaaataggagagggcaaccctttgccttcctacctcttgagaatgtacattattatccactttttgaaacttcttttaattgcttttttttaatttgtcttttcaaatagcataaccttgttcatccatttctgggaaccaaatttatcaatcaacagtgcctctaatctggctattaatacaaaaatgcctcctcaaaatatatatgttcgagtcttatctaaaacagaacccacaataaaaaagaagaaagaatacatataagcatttatataattctgagcaaccttgtgctttgtgaaaaaaatataatctaatgtcacatgctgtattctttttatttaacactggtgaaattataccattagagagaaagaggacagatcactgatcctaggatctagggatgttacagataagaaaacaaatgtgacaaagagctgtcacaaggaggatcttcaaggtcacagaatcactgtcttgatttcagtggtggttacatacatttaaatatgtgataaaatgttgttgaactatattcatatattgtaccaatgtcaaatgcttaattttggctctatagtataattatgcactaaataactatttggacaaagaaaatgatgtttacatcaaaggtgaggccatatttgttaggaacataacttaaaaaccattttggataactaatgaaaagccattttgtgtgccttggcatatcatgcctaagctgtcaccagatagatctaataagacctaagcctcagaagcaagcccctgcccagcaagcaggcagcacagataagagctaaacccaggacaggccatgatatgctaatgaactaccttcaaggtggtgttgctgacctagtgaaccagccccaagctgtgagccccaatagcacaaagctactgcccaaagaaattatacaaaaattggaactttgggaatggtgtgcaggatcgctctgctgtatgcctggaacacagcttctctatgttttgtattgataccagtctagaagcttccaaaactttctcactgaagaagattccccatgtgggacccctacagactcttttgcccaaacaactgcttccctcctggtgtgatatctgttttgcttttatgttagcataatattataaggaatgtttgtgtgaataaaccaaacatattttaaaagcaaatattgtatgcacatcctaattgctaaaaagtttacagctaatagtcccatgctctccacaatactggatccaaataagtcctaatttcaatgttgggcatctttacagagagaaagacattaaaaatgaagagacatgcagagagtgcaccatgccatcgtggagacagactgaagtgacacaactgttagtcaaagaggattaaggacttccagaagccaccaaaggaaggaggtatgaagtggtttctccctcagagtatccagaggagactaaaccaaccaacacctttttgcttaagacttcttgccttcaggactgtgagaaggtagcttcctattgttctaagccccagtatgtggcattttgttaaggtagagtcaagaaaccaataaaatgcagacagacaaaaggatagctgagttttccaggcccttccttcttatttttggttttgttggtggtggtggtggtggtggtgatggtggtggttttgtttatgttttgtttggggagttttttggggtttttttgggttttgtttttgttgttgttttgggggtttttgttgttgttgttgtttgcttttttgttttttgttttttgtttttttgagacagtgtttctctgtatagccctggctgtcctggagttccttctatctctaatgtctacatctcagaggggatcctctaatttcaaatgagcagtagctctccatttttagctcttatttattcatttatttacttacttacttattgtctgtagatgaaagaattttggagtgggaaagggttcatgagcccccagcaactaatgaggagctacagacaattgatgtttctggggaaaggagactcagtttctttgagagtatagcttctgatgggtcaaccatgttcctgtggctgatgtcacacccaggagtatgcagacaacagaaactggagttaatgagttgttttaaaaataaaaaagggcatgaagcttgggatagaaattaaggataaatacaattaaatacaggaaattctgaaagaattaataaaaacatttctttttttaaaaaaaaatccagaattagctatgcttcttcaaaattgcttctggagaactttacaagttaaataagttatattgtagaaaaggtagagaggagaatagtggaagagagagataaggagacttcaaaaggagtggagggagatagaggaggagaaagcagaagcaatggctgatagacacaggataagagggaacagaaaggagaaagaggaagccaggatgggtatttctttgcctatctgtgacttgcacatggtcttggcaattattgatgagttcaaggcttaattcttcacttgtgccaactcaacagagtctttctttcttataaccaggcccccagtatgctcatgtatgtatcaggtcctcttatctccttatagcaatcctgtttataactgggtaactttgtgaagggaaggaagtgcacactgagatgtgctacaactttttaatacaaaattttgaagagtttgtacaatgtatgtataattaataattaatattatgcactttagattttgatttcaactcaagatactaattctatatatatgggttaaatcaatatattaataagtttaatttcacatgcttatttttattgtggttttcgagacagggtttctctgtatagccctggctgtcctggaacccactttgtagaccaggctggcctcaaactcagaaacctacctgcctctgcctctgcctctgcctctgcctctgcctctgcctctgcctctgcctctgcctctgcctctgcctctgcctctgcctctgcctctgcctctgcctctgcctctgcctctgcctctgcctctgcctctgcctctgcctctgcctctgcctctgcctctgcctctgcctctgcctagtgctggaattaaaggtttgcgccaccacgcccggtgaaatttttaaactttatatatgtctcattctatttctatcagataggactgtgtagactgtgctaaactaataaatgtgccctcaaaagtaatcgcaagttgtattgttgttgttttgctttgctttgctttgctttgctttgctttgctttgctttgctttgctttgctttgctttgctttgctttgctttgctttgctttgctttgctttgctttgcttttttgttttgggtttttttccgggggagggagggtggagaaagaatcttactatgaagctctgactgtcctgggaactcactatatagatcaggcttgattcaactcatagagatctgccttcttctgcctcccaagtgctgggaataaaggcatacacctccatgcccagatagtgatcccaagttttagcaaaagtttctagacttgacattaatcgatggagatagacatgaattacacaaagaactaatgtggagtttacctgaatcatactctatactttatcagagattaaattaacatttaataatccagtgccaggctagaggcaccattcaatggcagtgtttgccatcatgcataggcttagtcttcagtgctgaaaggcattgggggcaatattactcattatacagatgagaaactgggaaagacttgcctcagattctctactgaaaggctgagtttgtggcttctagaaaatcttttactttcaatatttttaatgtataatttttttatttccactgattttattttttatttttaacatttataagaaataaatgcaataaaccaaatacatggacaaaaaaatacaagaatcatatgatcacctcaatggaaggaaaaaaaaagaaagaaaaagtctttgataagattcaacattcattctttttttattagatattttcttcatttacatttcaaatgctatccccaaagccccctataccttcccctgccctgctccccaacccacccactcctgctttctggccctggcattcctctgtactgaggcatatgatcttcaaaaaaccaagggcctctcctctcattggtggccgactattaggccatcttttgctacatatgcaactagagacacagctctgggggttactggttagttcatattgttagtcctcctatagagttgcagacccctttagctccttggatactttctctagttccttcattaggggccctgtgtcccatccaatagatgactgtgagcatccacttctgtatttgccaggcactggcatagcctcacgagaaagagagagctatgtcaggatcctgtcagtaaaatctttctggcatatgcaatagtatctgggtttggtggttgtatatgggatggatccccaagtggagcagtctctgaatggtccttccttccatctcagctccaaactttgtctctataactccttccatgggtattttgttccccattctaagaaggagtgaagaatccacactttggtcttccttcttcttgagtttcatatgttgcatcttggatattctaagtttctgggttaatatccacgtatcagtgagtgcatatcatgcgtgttattttgtgattagtttacctcactcaggatgatatcctccagatgcatccatttgcctaagaatttcattaattcactgtttttaattgctgaatagtactccattgtgtaaatgtaccacattttctgtatccattcctctgttgaggggcatctgggttctttccagcttctggctattataaataaggctgctatgagcatagcggagcatgtgtccttatcaagttggaacatcttctaggtatatgcccaggagaggaattgctggatcttccggtagtaccatcaacatgcattcttaataaaagccctagaacaaggaggactgtaggaaacatattccaacataataaaggttatgtatgacaaactcatgaccaatatcatcctaaatgaatgaaaccattaataagctccattaaaatcagaggactgcccactatccctacttctcatccataatgagattgaagcattagctggagcaataaggcaagagaagggatacaaatgggaaaatattaagtcaaattgttttcaattgaagattatattatcttatacccaatgacctcaaattttgactagaaaaattgtagaaattatcaataatttcagcaaagtgttatgatgcaccacatccttattcttctccccagcttctgcttgcttctctcttcttgctcttcatcctttctgtccttccatctgcctgcactcttgtctcaagactgagtgcagcgtgtaactctcctgtgactgagtatctcacaaaacgttctacctgccaaacctggatgagccctttgtctttctgaagctatgaggctctctacatagactcaagaaggaaatgacagggaggaggtaataatgaagtggggaaggctgacattagcattgctcctgtgtggctccttaatttctcatacttcacactgagatgttattaactgtgactcataggtgaagaagccagagctaaggttctcatatttgagtgttatagaatgagtagagcagtagttctcaaactatgggtcatgactcctttatgggtcaaactaccctttcacacaggttgcatatcagatatcctaattttatatacatatatatatgcatatgtatatatatatatttcacaacagtaggaaaattatttagtaatcattttatagttgtgggtcatggcaacatgaggaactgtattaaagggttgcagcattaggaatgttgagacccactgtaatagagaatgaggcttaaggcagggctataaagcccaatggaccatgtgccttttccaacatttgccacatggtaagctctgtatagactttttaaagaacattggtttgtaattttaaatggataagggtcttcactgtctatcacccatctatataataaatacataagttttgattccaccatggattcaaatgcaaaaatcctcaacctaagacatagcagtgaaacattgatgaccaaataggaaatccatgtagagaccttctatcttctgatggctccacaggcaccatcttgcaacagagttctactttgctaccagtaatgaatacagtgtctcaactcctgccattgaatcttcaggaagcccctgaaatgacttgtactacaccatttcttaaagacagaaaagctaagacttagagggaataaatgtcatgcctgagatcatgcaaccaattaagtccaacttggcctgatcaagaggcacaattcaaaagcaatgttgttccttcactagctcttgtgtatggttgctgattccggaagcaaagtatcagtgaatatccctagtgggaaaagacttggaaatcaaatgtctcatttaacagattaggagatgaaacggtagactctgtgtagttgtacacccctgtgatcccatcgctaggaagactgaggcaggaagtcctcgagctcaaaccagcttaggctacacagagaaactatctaaaaaataattactaactacttaataggagattggatgttaagatctggtcactaagaggcagaattgagattcgaagccagtattttctacctggtatgttttaaattgcagtaaggatctaagtgtagatatataataataagattctattgatctctgcaacaacagagagtgttagatttgtttggaaaaaaatattatcagccaacatcttctaccatttcagtatagcacagagtacccacccatatctccccacccatcccccataccagactggttattgattttcatggtgactggcctgagaagattaaaaaaagtaatgctaccttattgggagtgtcccatggaccaagatagcaactgtcatagctaccgtcacactgctttgatcaagaagaccctttgaggaactgaaaacagaaccttaggcacatctgttgctttcgctcccatcctcctccaacagcctgggtggtgcactccacaccctttcaagtttccaaagcctcatacacctgctccctaccccagcacctggccaaggctgtatccagcactgggatgaaaatgataccccacctccatcttgtttgatattactctatctcaagccccaggttagtccccagtcccaatgcttttgcacagtcaaaactcaacttggaataatcagtatccttgaagagttctgatatggtcactgggcccatataccatgtaagacatgtggaaaagatgtttcatggggcccagacacgttctagaagtacctgagagtggcaaaaaatagttgtgctaaatagtttggccatctttaggctgagagactaggaaatacagcgatggactatatcagcattgcaggatagttgtcagtaaacaccccacaacccataacagaagtattctcttctttctatatcccttttccatccatgtagatggctgtcttcatatttgttctagacggccggcc

SEQ ID NO: 96 - DNA, 4638 bp, Artificial
  pSELECT-IGKV1-39/J-Ck
gcggccgcaataaaatatctttattttcattacatctgtgtgttggttttttgtgtgaatcgtaactaacatacgctctccatcaaaacaaaacgaaacaaaacaaactagcaaaataggctgtccccagtgcaagtgcaggtgccagaacatttctctatcgaaggatctgcgatcgctccggtgcccgtcagtgggcagagcgcacatcgcccacagtccccgagaagttggggggaggggtcggcaattgaacgggtgcctagagaaggtggcgcggggtaaactgggaaagtgatgtcgtgtactggctccgcctttttcccgagggtgggggagaaccgtatataagtgcagtagtcgccgtgaacgttctttttcgcaacgggtttgccgccagaacacagctgaagcttcgaggggctcgcatctctccttcacgcgcccgccgccctacctgaggccgccatccacgccggttgagtcgcgttctgccgcctcccgcctgtggtgcctcctgaactgcgtccgccgtctaggtaagtttaaagctcaggtcgagaccgggcctttgtccggcgctcccttggagcctacctagactcagccggctctccacgctttgcctgaccctgcttgctcaactctacgtctttgtttcgttttctgttctgcgccgttacagatccaagctgtgaccggcgcctacctgagatcaccggcgtgtcgacgccaccatggacatgagagtgcccgcccagctcctggggctcctgctactctggctccgaggtaaggatggagaacactaggaatttactcagccagtgtgctcagtactgactggaacttcagggaagttctctgataacatgattaatagtaagaatatttgtttttatgtttccaatctcaggtgccagatgtgacatccagatgacccagagccccagcagcctgagcgccagcgtgggcgacagagtgaccatcacctgcagagccagccagagcatcagcagctacctgaactggtatcagcagaagcccggcaaggcccccaagctgctgatctacgccgccagctccctgcagagcggcgtgcccagcagattcagcggcagcggctccggcaccgacttcaccctgaccatcagcagcctgcagcccgaggacttcgccacctactactgccagcagagctacagcaccccccccaccttcggccagggcaccaaggtggagatcaagagagccgacgccgctcccaccgtgtccatcttcccccccagcatggaacagctgacctctggcggagccaccgtggtctgcttcgtgaacaacttctaccccagagacatcagcgtgaagtggaagatcgacggcagcgagcagagggacggcgtgctggacagcgtgaccgaccaggacagcaaggactccacctacagcatgagcagcaccctgagcctgaccaaggtggagtacgagaggcacaacctgtacacctgcgaggtggtgcacaagaccagctccagccccgtggtcaagtccttcaaccggaacgagtgttgagctagctggccagacatgataagatacattgatgagtttggacaaaccacaactagaatgcagtgaaaaaaatgctttatttgtgaaatttgtgatgctattgctttatttgtaaccattataagctgcaataaacaagttaacaacaacaattgcattcattttatgtttcaggttcagggggaggtgtgggaggttttttaaagcaagtaaaacctctacaaatgtggtatggaattctaaaatacagcatagcaaaactttaacctccaaatcaagcctctacttgaatccttttctgagggatgaataaggcataggcatcaggggctgttgccaatgtgcattagctgtttgcagcctcaccttctttcatggagtttaagatatagtgtattttcccaaggtttgaactagctcttcatttctttatgttttaaatgcactgacctcccacattccctttttagtaaaatattcagaaataatttaaatacatcattgcaatgaaaataaatgttttttattaggcagaatccagatgctcaaggcccttcataatatcccccagtttagtagttggacttagggaacaaaggaacctttaatagaaattggacagcaagaaagcgagcttctagcgaattctcgactcattcctttgccctcggacgagtgctggggcgtcggtttccactatcggcgagtacttctacacagccatcggtccagacggccgcgcttctgcgggcgatttgtgtacgcccgacagtcccggctccggatcggacgattgcgtcgcatcgaccctgcgcccaagctgcatcatcgaaattgccgtcaaccaagctctgatagagttggtcaagaccaatgcggagcatatacgcccggagccgcggcgatcctgcaagctccggatgcctccgctcgaagtagcgcgtctgctgctccatacaagccaaccacggcctccagaagaagatgttggcgacctcgtattgggaatccccgaacatcgcctcgctccagtcaatgaccgctgttatgcggccattgtccgtcaggacattgttggagccgaaatccgcgtgcacgaggtgccggacttcggggcagtcctcggcccaaagcatcagctcatcgagagcctgcgcgacggacgcactgacggtgtcgtccatcacagtttgccagtgatacacatggggatcagcaatcgcgcatatgaaatcacgccatgtagtgtattgaccgattccttgcggtccgaatgggccgaacccgctcgtctggctaagatcggccgcagcgatcgcatccatgagctccgcgacgggttgcagaacagcgggcagttcggtttcaggcaggtcttgcaacgtgacaccctgtgcacggcgggagatgcaataggtcaggctctcgctgaattccccaatgtcaagcacttccggaatcgggagcgcggccgatgcaaagtgccgataaacataacgatctttgtagaaaccatcggcgcagctatttacccgcaggacatatccacgccctcctacatcgaagctgaaagcacgagattcttcgccctccgagagctgcatcaggtcggagacgctgtcgaacttttcgatcagaaacttctcgacagacgtcgcggtgagttcaggctttttcatgatggccctcctatagtgagtcgtattatactatgccgatatactatgccgatgattaattgtcaaaacagcgtggatggcgtctccagcttatctgacggttcactaaacgagctctgcttatatagacctcccaccgtacacgcctaccgcccatttgcgtcaatggggcggagttgttacgacattttggaaagtcccgttgatttactagtcaaaacaaactcccattgacgtcaatggggtggagacttggaaatccccgtgagtcaaaccgctatccacgcccattgatgtactgccaaaaccgcatcatcatggtaatagcgatgactaatacgtagatgtactgccaagtaggaaagtcccataaggtcatgtactgggcataatgccaggcgggccatttaccgtcattgacgtcaatagggggcgtacttggcatatgatacacttgatgtactgccaagtgggcagtttaccgtaaatactccacccattgacgtcaatggaaagtccctattggcgttactatgggaacatacgtcattattgacgtcaatgggcgggggtcgttgggcggtcagccaggcgggccatttaccgtaagttatgtaacgcctgcaggttaattaagaacatgtgagcaaaaggccagcaaaaggccaggaaccgtaaaaaggccgcgttgctggcgtttttccataggctccgcccccctgacgagcatcacaaaaatcgacgctcaagtcagaggtggcgaaacccgacaggactataaagataccaggcgtttccccctggaagctccctcgtgcgctctcctgttccgaccctgccgcttaccggatacctgtccgcctttctcccttcgggaagcgtggcgctttctcatagctcacgctgtaggtatctcagttcggtgtaggtcgttcgctccaagctgggctgtgtgcacgaaccccccgttcagcccgaccgctgcgccttatccggtaactatcgtcttgagtccaacccggtaagacacgacttatcgccactggcagcagccactggtaacaggattagcagagcgaggtatgtaggcggtgctacagagttcttgaagtggtggcctaactacggctacactagaagaacagtatttggtatctgcgctctgctgaagccagttaccttcggaaaaagagttggtagctcttgatccggcaaacaaaccaccgctggtagcggtggtttttttgtttgcaagcagcagattacgcgcagaaaaaaaggatctcaagaagatcctttgatcttttctacggggtctgacgctcagtggaacgaaaactcacgttaagggattttggtcatggctagttaattaacatttaaatca

SEQ ID NO: 97 - DNA, 5349 bp, Artificial
  pSelect-IGVL2-14/J-Ck
gcggccgcaataaaatatctttattttcattacatctgtgtgttggttttttgtgtgaatcgtaactaacatacgctctccatcaaaacaaaacgaaacaaaacaaactagcaaaataggctgtccccagtgcaagtgcaggtgccagaacatttctctatcgaaggatctgcgatcgctccggtgcccgtcagtgggcagagcgcacatcgcccacagtccccgagaagttggggggaggggtcggcaattgaacgggtgcctagagaaggtggcgcggggtaaactgggaaagtgatgtcgtgtactggctccgcctttttcccgagggtgggggagaaccgtatataagtgcagtagtcgccgtgaacgttctttttcgcaacgggtttgccgccagaacacagctgaagcttcgaggggctcgcatctctccttcacgcgcccgccgccctacctgaggccgccatccacgccggttgagtcgcgttctgccgcctcccgcctgtggtgcctcctgaactgcgtccgccgtctaggtaagtttaaagctcaggtcgagaccgggcctttgtccggcgctcccttggagcctacctagactcagccggctctccacgctttgcctgaccctgcttgctcaactctacgtctttgtttcgttttctgttctgcgccgttacagatccaagctgtgaccggcgcctacctgagatcaccggcgtgtcgacgccaccatggacatgagagtgcccgcccagctcctggggctcctgctactctggctccgaggtaaggatggagaacactaggaatttactcagccagtgtgctcagtactgactggaacttcagggaagttctctgataacatgattaatagtaagaatatttgtttttatgtttccaatctcaggtgccagatgtcagtctgccctgacccagcccgcctctgtgtctggcagccctggccagagcatcaccatcagctgcaccggcaccagcagcgacgtgggcggctacaactacgtgtcctggtatcagcagcaccccggcaaggcccccaagctgatgatctacgaggtgtccaacagacccagcggcgtgagcaacagattcagcggcagcaagagcggcaacaccgccagcctgaccatcagcggcctccaggctgaggacgaggccgactactactgcagcagctacaccagcagctccaccctggtgtttggcggcggaacaaagctgaccgtgctgagagccgacgccgctcccaccgtgtccatcttcccccccagcatggaacagctgacctctggcggagccaccgtggtctgcttcgtgaacaacttctaccccagagacatcagcgtgaagtggaagatcgacggcagcgagcagagggacggcgtgctggacagcgtgaccgaccaggacagcaaggactccacctacagcatgagcagcaccctgagcctgaccaaggtggagtacgagaggcacaacctgtacacctgcgaggtggtgcacaagaccagctccagccccgtggtcaagtccttcaaccggaacgagtgttgagctagctggccagacatgataagatacattgatgagtttggacaaaccacaactagactgactcagcctgcctccgtgtctgggtctcctggacagtcgatcaccatctcctgcactggaaccagcagtgacgttggtggttataactatgtctcctggtaccaacagcacccaggcaaagcccccaaactcatgatttatgaggtcagtaatcggccctcaggggtttctaatcgcttctctggctccaagtctggcaacacggcctccctgaccatctctgggctccaggctgaggacgaggctgattattactgcagctcatatacaagcagcagcactctcgtattcggcggagggaccaagctgaccgtcctacgggctgatgctgcaccaactgtatccatcttcccaccatccatggaacagttaacatctggaggtgccacagtcgtgtgcttcgtgaacaacttctatcccagagacatcagtgtcaagtggaagattgatggcagtgaacaacgagatggtgtcctggacagtgttactgatcaggacagcaaagacagcacgtacagcatgagcagcaccctctcgttgaccaaggttgaatatgaaaggcataacctctatacctgtgaggttgttcataagacatcatcctcacccgtcgtcaagagcttcaacaggaatgagtgttaggctagctggccagacatgataagatacattgatgagtttggacaaaccacaactagaatgcagtgaaaaaaatgctttatttgtgaaatttgtgatgctattgctttatttgtaaccattataagctgcaataaacaagttaacaacaacaattgcattcattttatgtttcaggttcagggggaggtgtgggaggttttttaaagcaagtaaaacctctacaaatgtggtatggaattctaaaatacagcatagcaaaactttaacctccaaatcaagcctctacttgaatccttttctgagggatgaataaggcataggcatcaggggctgttgccaatgtgcattagctgtttgcagcctcaccttctttcatggagtttaagatatagtgtattttcccaaggtttgaactagctcttcatttctttatgttttaaatgcactgacctcccacattccctttttagtaaaatattcagaaataatttaaatacatcattgcaatgaaaataaatgttttttattaggcagaatccagatgctcaaggcccttcataatatcccccagtttagtagttggacttagggaacaaaggaacctttaatagaaattggacagcaagaaagcgagcttctagcgaattctcgactcattcctttgccctcggacgagtgctggggcgtcggtttccactatcggcgagtacttctacacagccatcggtccagacggccgcgcttctgcgggcgatttgtgtacgcccgacagtcccggctccggatcggacgattgcgtcgcatcgaccctgcgcccaagctgcatcatcgaaattgccgtcaaccaagctctgatagagttggtcaagaccaatgcggagcatatacgcccggagccgcggcgatcctgcaagctccggatgcctccgctcgaagtagcgcgtctgctgctccatacaagccaaccacggcctccagaagaagatgttggcgacctcgtattgggaatccccgaacatcgcctcgctccagtcaatgaccgctgttatgcggccattgtccgtcaggacattgttggagccgaaatccgcgtgcacgaggtgccggacttcggggcagtcctcggcccaaagcatcagctcatcgagagcctgcgcgacggacgcactgacggtgtcgtccatcacagtttgccagtgatacacatggggatcagcaatcgcgcatatgaaatcacgccatgtagtgtattgaccgattccttgcggtccgaatgggccgaacccgctcgtctggctaagatcggccgcagcgatcgcatccatgagctccgcgacgggttgcagaacagcgggcagttcggtttcaggcaggtcttgcaacgtgacaccctgtgcacggcgggagatgcaataggtcaggctctcgctgaattccccaatgtcaagcacttccggaatcgggagcgcggccgatgcaaagtgccgataaacataacgatctttgtagaaaccatcggcgcagctatttacccgcaggacatatccacgccctcctacatcgaagctgaaagcacgagattcttcgccctccgagagctgcatcaggtcggagacgctgtcgaacttttcgatcagaaacttctcgacagacgtcgcggtgagttcaggctttttcatgatggccctcctatagtgagtcgtattatactatgccgatatactatgccgatgattaattgtcaaaacagcgtggatggcgtctccagcttatctgacggttcactaaacgagctctgcttatatagacctcccaccgtacacgcctaccgcccatttgcgtcaatggggcggagttgttacgacattttggaaagtcccgttgatttactagtcaaaacaaactcccattgacgtcaatggggtggagacttggaaatccccgtgagtcaaaccgctatccacgcccattgatgtactgccaaaaccgcatcatcatggtaatagcgatgactaatacgtagatgtactgccaagtaggaaagtcccataaggtcatgtactgggcataatgccaggcgggccatttaccgtcattgacgtcaatagggggcgtacttggcatatgatacacttgatgtactgccaagtgggcagtttaccgtaaatactccacccattgacgtcaatggaaagtccctattggcgttactatgggaacatacgtcattattgacgtcaatgggcgggggtcgttgggcggtcagccaggcgggccatttaccgtaagttatgtaacgcctgcaggttaattaagaacatgtgagcaaaaggccagcaaaaggccaggaaccgtaaaaaggccgcgttgctggcgtttttccataggctccgcccccctgacgagcatcacaaaaatcgacgctcaagtcagaggtggcgaaacccgacaggactataaagataccaggcgtttccccctggaagctccctcgtgcgctctcctgttccgaccctgccgcttaccggatacctgtccgcctttctcccttcgggaagcgtggcgctttctcatagctcacgctgtaggtatctcagttcggtgtaggtcgttcgctccaagctgggctgtgtgcacgaaccccccgttcagcccgaccgctgcgccttatccggtaactatcgtcttgagtccaacccggtaagacacgacttatcgccactggcagcagccactggtaacaggattagcagagcgaggtatgtaggcggtgctacagagttcttgaagtggtggcctaactacggctacactagaagaacagtatttggtatctgcgctctgctgaagccagttaccttcggaaaaagagttggtagctcttgatccggcaaacaaaccaccgctggtagcggtggtttttttgtttgcaagcagcagattacgcgcagaaaaaaaggatctcaagaagatcctttgatcttttctacggggtctgacgctcagtggaacgaaaactcacgttaagggattttggtcatggctagttaattaacatttaaatca

SEQ ID NO: 98 - DNA, 6772 bp, Artificial
  MV1043
cttgatttgggtgatggttcacgtagtgggccatcgccctgatagacggtttttcgccctttgacgttggagtccacgttctttaatagtggactcttgttccaaactggaacaacactcaactctatctcgggctattcttttgatttataagggattttgccgatttcggtctattggttaaaaaatgagctgatttaacaaaaatttaacgcgaattttaacaaaatattaacgtttacaattttatggtgcagtctcagtacaatctgctctgatgccgcatagttaagccagccccgacacccgccaacacccgctgacgcgccctgacgggcttgtctgctcccggcatccgcttacagacaagctgtgaccgtctccgggagctgcatgtgtcagaggttttcaccgtcatcaccgaaacgcgcgagacgaaagggcctcgtgatacgcctatttttataggttaatgtcatgataataatggtttcttagacgtcaggtggcacttttcggggaaatgtgcgcggaacccctatttgtttatttttctaaatacattcaaatatgtatccgctcatgagacaataaccctgataaatgcttcaataatattgaaaaaggaagagtatgagtattcaacatttccgtgtcgcccttattcccttttttgcggcattttgccttcctgtttttgctcacccagaaacgctggtgaaagtaaaagatgctgaagatcagttgggtgcccgagtgggttacatcgaactggatctcaacagcggtaagatccttgagagttttcgccccgaagaacgttttccaatgatgagcacttttaaagttctgctatgtggcgcggtattatcccgtattgacgccgggcaagagcaactcggtcgccgcatacactattctcagaatgacttggttgagtactcaccagtcacagaaaagcatcttacggatggcatgacagtaagagaattatgcagtgctgccataaccatgagtgataacactgcggccaacttacttctgacaacgatcggaggaccgaaggagctaaccgcttttttgcacaacatgggggatcatgtaactcgccttgatcgttgggaaccggagctgaatgaagccataccaaacgacgagcgtgacaccacgatgcctgtagcaatggcaacaacgttgcgcaaactattaactggcgaactacttactctagcttcccggcaacaattaatagactggatggaggcggataaagttgcaggaccacttctgcgctcggcccttccggctggctggtttattgctgataaatctggagccggtgagcgtgggtctcgcggtatcattgcagcactggggccagatggtaagccctcccgtatcgtagttatctacacgacggggagtcaggcaactatggatgaacgaaatagacagatcgctgagataggtgcctcactgattaagcattggtaactgtcagaccaagtttactcatatatactttagattgatttaaaacttcatttttaatttaaaaggatctaggtgaagatcctttttgataatctcatgaccaaaatcccttaacgtgagttttcgttccactgagcgtcagaccccgtagaaaagatcaaaggatcttcttgagatcctttttttctgcgcgtaatctgctgcttgcaaacaaaaaaaccaccgctaccagcggtggtttgtttgccggatcaagagctaccaactctttttccgaaggtaactggcttcagcagagcgcagataccaaatactgttcttctagtgtagccgtagttaggccaccacttcaagaactctgtagcaccgcctacatacctcgctctgctaatcctgttaccagtggctgctgccagtggcgataagtcgtgtcttaccgggttggactcaagacgatagttaccggataaggcgcagcggtcgggctgaacggggggttcgtgcatacagcccagcttggagcgaacgacctacaccgaactgagatacctacagcgtgagctatgagaaagcgccacgcttcccgaagggagaaaggcggacaggtatccggtaagcggcagggtcggaacaggagagcgcacgagggagcttccagggggaaacgcctggtatctttatagtcctgtcgggtttcgccacctctgacttgagcgtcgatttttgtgatgctcgtcaggggggcggagcctatggaaaaacgccagcaacgcggcctttttacggttcctggccttttgctggccttttgctcacatgttctttcctgcgttatcccctgattctgtggataaccgtattaccgcctttgagtgagctgataccgctcgccgcagccgaacgaccgagcgcagcgagtcagtgagcgaggaagcggaagagcgcccaatacgcaaaccgcctctccccgcgcgttggccgattcattaatgcagctggcacgacaggtttcccgactggaaagcgggcagtgagcgcaacgcaattaatgtgagttagctcactcattaggcaccccaggctttacactttatgcttccggctcgtatgttgtgtggaattgtgagcggataacaatttcacacaggaaacagctatgaccatgattacgccaagctttggagccttttttttggagattttcaacgtgaaaaaattattattcgcaattcctttagttgttcctttctattctcacagtgcacagatccaaatgacccagtctccatcctccctgtctgcatctgtaggagacagagtcaccatcacttgccgggcaagtcagagcattagcagctacttaaattggtatcagcagaaaccagggaaagcccctaagctcctgatctatgctgcatccagtttgcaaagtggggtcccatcaaggttcagtggcagtggatctgggacagatttcactctcaccatcagcagtctgcaacctgaagattttgcaacttactactgtcaacagagttacagtacccctccaacgttcggccaagggaccaagctcgagatcaaacgtactgtggctgcaccatctgtcttcatcttcccgccatctgatgagcagttgaaatctggaactgcctctgttgtgtgcctgctgaataacttctatcccagagaggccaaagtacagtggaaggtggataacgccctccaatcgggtaactcccaggagagtgtcacagagcaggacagcaaggacagcacctacagcctcagcagcaccctgacgctgagcaaagcagactacgagaaacacaaagtctacgcctgcgaagtcacccatcagggcctgagctcgcccgtcacaaagagcttcaacaggggagagtgttagtaaggcgcgccaattctatttcaaggagacagtcataatgaaatacctattgcctacggcagccgctggattgttattactcgcggcccagccggccatggcgatgcctgcttgccgaatatcatggtggaaaatggccgcttttctggattcatcgactgtggccggctgggtgtggcggaccgctatcaggacatagcgttggctacccgtgatattgctgaagagcttggcggcgaatgggctgaccgcttcctcgtgctttacggtatcgccgctcccgattcgcagcgcatcgccttctatcgccttcttgacgagttcttctgagcgggactctggggttcggtgctacgagatttcgattccaccgccgccttctatgaaaggttgggcttcggaatcgttttccgggacgccggctggatgatcctccagcgcggggatctcatgctggagttcttcgcccaccccaacttgtttattgcagcttataatggttacaaataaagcaatagcatcacaaatttcacaaataaagcatttttttcactgcattctagttgtggtttgtccaaactcatcaatgtatcttatcatgtctgtataccgtcgacctctagctagagcttggcgtaatcatggtcatagctgtttcctgtgtgaaattgttatccgctcacaattccacacaacatacgagccggaagcataaagtgtaaagcctggggtgcctaatgagtgagctaactcacattaattgcgttgcgctcactgcccgctttccagtcgggaaacctgtcgtgccagaattgcatgaagaatctgcttagggttaggcgttttgcgctgcttcgctaggtggtcaatattggccattagccatattattcattggttatatagcataaatcaatattggctattggccattgcatacgttgtatccatatcataatatgtacatttatattggctcatgtccaacattaccgccatgttgacattgattattgactagttattaatagtaatcaattacggggtcattagttcatagcccatatatggagttccgcgttacataacttacggtaaatggcccgcctggctgaccgcccaacgacccccgcccattgacgtcaataatgacgtatgttcccatagtaacgccaatagggactttccattgacgtcaatgggtggagtatttacggtaaactgcccacttggcagtacatcaagtgtatcatatgccaagtacgccccctattgacgtcaatgacggtcaccgtctcaagcgcctccaccaagggcccatcggtcttccccctggcaccctcctccaagagcacctctgggggcacagcggccctgggctgcctggtcaaggactacttccccgaaccggtgacggtgtcgtggaactcaggcgccctgaccagcggcgtccacaccttcccggctgtcctacagtcctcaggactctactccctcagcagcgtagtgaccgtgccctccagcagcttgggcacccagacctacatctgcaacgtgaatcacaagcccagcaacaccaaggtggacaagaaagttgagcccaaatcttgtgcggccgcacatcatcatcaccatcacggggccgcagaacaaaaactcatctcagaagaggatctgaatggggccgcatagactgttgaaagttgtttagcaaaacctcatacagaaaattcatttactaacgtctggaaagacgacaaaactttagatcgttacgctaactatgagggctgtctgtggaatgctacaggcgttgtggtttgtactggtgacgaaactcagtgttacggtacatgggttcctattgggcttgctatccctgaaaatgagggtggtggctctgagggtggcggttctgagggtggcggttctgagggtggcggtactaaacctcctgagtacggtgatacacctattccgggctatacttatatcaaccctctcgacggcacttatccgcctggtactgagcaaaaccccgctaatcctaatccttctcttgaggagtctcagcctcttaatactttcatgtttcagaataataggttccgaaataggcagggtgcattaactgtttatacgggcactgttactcaaggcactgaccccgttaaaacttattaccagtacactcctgtatcatcaaaagccatgtatgacgcttactggaacggtaaattcagagactgcgctttccattctggctttaatgaggatccattcgtttgtgaatatcaaggccaatcgtctgacctgcctcaacctcctgtcaatgctggcggcggctctggtggtggttctggtggcggctctgagggtggcggctctgagggtggcggctctgagggtggcggttctgagggtggcggctctgagggtggcggttccggtggcggctccggttccggtgattttgattatgaaaaaatggcaaacgctaataagggggctatgaccgaaaatgccgatgaaaacgcgctacagtctgacgctaaaggcaaacttgattctgtcgctactgattacggtgctgctatcgatggtttcattggtgacgtttccggccttgctaatggtaatggtgctactggtgattttgctggctctaattcccaaatggctcaagtcggtgacggtgataattcacctttaatgaataatttccgtcaatatttaccttctttgcctcagtcggttgaatgtcgcccttatgtctttggcgctggtaaaccatatgaattttctattgattgtgacaaaataaacttattccgtggtgtctttgcgtttcttttatatgttgccacctttatgtatgtattttcgacgtttgctaacatactgcgtaataaggagtcttaataagaattcactggccgtcgttttacaacgtcgtgactgggaaaaccctggcgttacccaacttaatcgccttgcagcacatccccctttcgccagctggcgtaatagcgaagaggcccgcaccgatcgcccttcccaacagttgcgcagcctgaatggcgaatggcgcctgatgcggtattttctccttacgcatctgtgcggtatttcacaccgcatacgtcaaagcaaccatagtacgcgccctgtagcggcgcattaagcgcggcgggtgtggtggttacgcgcagcgtgaccgctacacttgccagcgccttagcgcccgctcctttcgctttcttcccttcctttctcgccacgttcgccggctttccccgtcaagctctaaatcgggggctccctttagggttccgatttagtgctttacggcacctcgaccccaaaaaa

SEQ ID NO: 99 - DNA, 10293 bp, Artificial
  MV1057
tactcttcctttttcaatattattgaagcatttatcagggttattgtctcatgagcggatacatatttgaatgtatttagaaaaataaacaaataggggttccgcgcacatttccccgaaaagtgccacctgacgtcgacggatcgggagatctcccgatcccctatggtgcactctcagtacaatctgctctgatgccgcatagttaagccagtatctgctccctgcttgtgtgttggaggtcgctgagtagtgcgcgagcaaaatttaagctacaacaaggcaaggcttgaccgacaattgcatgaagaatctgcttagggttaggcgttttgcgctgcttcgctaggtggtcaatattggccattagccatattattcattggttatatagcataaatcaatattggctattggccattgcatacgttgtatccatatcataatatgtacatttatattggctcatgtccaacattaccgccatgttgacattgattattgactagttattaatagtaatcaattacggggtcattagttcatagcccatatatggagttccgcgttacataacttacggtaaatggcccgcctggctgaccgcccaacgacccccgcccattgacgtcaataatgacgtatgttcccatagtaacgccaatagggactttccattgacgtcaatgggtggagtatttacggtaaactgcccacttggcagtacatcaagtgtatcatatgccaagtacgccccctattgacgtcaatgacggtaaatggcccgcctggcattatgcccagtacatgaccttatgggactttcctacttggcagtacatctacgtattagtcatcgctattaccatggtgatgcggttttggcagtacatcaatgggcgtggatagcggtttgactcacggggatttccaagtctccaccccattgacgtcaatgggagtttgttttggcaccaaaatcaacgggactttccaaaatgtcgtaacaactccgccccattgacgcaaatgggcggtaggcgtgtacggtgggaggtctatataagcagagctcgtttagtgaaccgtcagatcgcctggagacgccatccacgctgttttgacctccatagaagacaccgggaccgatccagcctccgcggccgggaacggtgcattggaagcttggtaccggtgaattggccggcccgcgccgtcgaggttatcgatccgaccgacgcgttcgcgagaggccgcaattccctagccaccatgggatggagctgtatcatcctcttcttggtactgctgctggcccagccggccatggggcggagaatgggcggaactgggcggagttaggggcgggatgggcggagttaggggcgggactatggttgctgactaattgagatgcggatccgctggcacgacaggtttcccgactggaaagcgggcagtgagcgcaacgcaattaatgtgagttagctcactcattaggcaccccaggctttacactttatgcttccggctcgtatgttgtgtggaattgtgagcggataacaatttcacacaggaaacagctatgaccatgattacgccaagcttgggctgcaggttctttccgcctcagaagccatagagcccaccgcatccccagcatgcctgctattgtcttcccaatcctcccccttgctgtcctgccccaccccaccccccagaatagaatgacacctactcagacaatgcgatgcaatttcctcattttattaggaaaggacagtgggagtggcaccttccagggtcaaggaaggcacgggggaggggcaaacaacagatggctggcaactagaaggcacagtcgaggctgatcagcgagctctagatcatcgatgcatggggtcgtgcgctcctttcggtcgggcgctgcgggtcgtggggcgggcgtcaggcaccgggcttgcgggtcatgcaccaggtgcgcggtccttcgggcacctcgacgtcggcggtgacggtgaagccgagccgctcgtagaaggggaggttgcggggcgcggaggtctccaggaaggcgggcaccccggcgcgctcggccgcctccactccggggagcacgacggcgctgcccagacccttgccctggtggtcgggcgagacgccgacggtggccaggaaccacgcgggctccttgggccggtgcggcgccaggaggccttccatctgttgctgcgcggccagccgggaaccgctcaactcggccatgcgcgggccgatctcggcgaacaccgcccccgcttcgacgctctccggcgtggtccagaccgccaccgcggcgccgtcgtccgcgacccacaccttgccgatgtcgagcccgacgcgcgtgaggaagagttcttgcagctcggtcaccgtctccagtgctagcaccaagggcccatcggtcttccccctggcaccctcctccaagagcacctctgggggcacagcggccctgggctgcctggtcaaggactacttccccgaaccggtgacggtgtcgtggaactcaggcgccctgaccagcggcgtgcacaccttcccggctgtcctacagtcctcaggactctactccctcagcagcgtcgtgaccgtgccctccagcagcttgggcacccagacctacatctgcaacgtgaatcacaagcccagcaacaccaaggtggacaagagagttggtgagaggccagcacagggagggagggtgtctgctggaagccaggctcagcgctcctgcctggacgcatcccggctatgcagtcccagtccagggcagcaaggcaggccccgtctgcctcttcacccggaggcctctgcccgccccactcatgctcagggagagggtcttctggctttttccccaggctctgggcaggcacaggctaggtgcccctaacccaggccctgcacacaaaggggcaggtgctgggctcagacctgccaagagccatatccgggaggaccctgcccctgacctaagcccaccccaaaggccaaactctccactccctcagctcggacaccttctctcctcccagattccagtaactcccaatcttctctctgcagagcccaaatcttgtgacaaaactcacacatgcccaccgtgcccagcacctgaactcctggggggaccgtcagtcttcctcttccccccaaaacccaaggacaccctcatgatctcccggacccctgaggtcacatgcgtggtggtggacgtgagccacgaagaccctgaggtcaagttcaactggtacgtggacggcgtggaggtgcataatgccaagacaaagccgcgggaggagcagtacaacagcacgtaccgtgtggtcagcgtcctcaccgtcctgcaccaggactggctgaatggcaaggagtacaagtgcaaggtctccaacaaagccctcccagcccccatcgagaaaaccatctccaaagccaaagggcagccccgagaaccacaggtgtacaccctgcccccatcccgggaggagatgaccaagaaccaggtcagcctgacctgcctggtcaaaggcttctatcccagcgacatcgccgtggagtgggagagcaatgggcagccggagaacaactacaagaccacgcctcccgtgctggactccgacggctccttcttcctctatagcaagctcaccgtggacaagagcaggtggcagcaggggaacgtcttctcatgctccgtgatgcatgaggctctgcacaaccactacacgcagaagagcctctccctgtctccgggtaaatgagtttaacggatcttaattaatccgagctcggtaccaagcttaagtttaaaccgctgatcagcctcgactgtgccttctagttgccagccatctgttgtttgcccctcccccgtgccttccttgaccctggaaggtgccactcccactgtcctttcctaataaaatgaggaaattgcatcgcattgtctgagtaggtgtcattctattctggggggtggggtggggcaggacagcaagggggaggattgggaagacaatagcaggcatgctggggatgcggtgggctctatggcttctgaggcggaaagaaccagctggggctctagggggtatccccacgcgccctgtagcggcgcattaagcgcggcgggtgtggtggttacgcgcagcgtgaccgctacacttgccagcgcctagcgcccgctcctttcgctttcttcccttcctttctcgccacgttcgccggctttccccgtcaagctctaaatcgggggctccctttagggttccgatttagtgctttacggcacctcgaccccaaaaaacttgattagggtgatggttcacgtagtgggccatcgccctgatagacggtttttcgccctttgacgttggagtccacgttctttaatagtggactcttgttccaaactggaacaacactcaaccctatctcggtctattcttttgatttataagggattttgccgatttcggcctattggttaaaaaatgagctgatttaacaaaaatttaacgcgaattaattctgtggaatgtgtgtcagttagggtgtggaaagtccccaggctccccagcaggcagaagtatgcaaagcatgcatctcaattagtcagcaaccaggtgtggaaagtccccaggctccccagcaggcagaagtatgcaaagcatgcatctcaattagtcagcaaccatagtcccgcccctaactccgcccatcccgcccctaactccgcccagttccgcccattctccgccccatggctgactaattttttttatttatgcagaggccgaggccgcctctgcctctgagctattccagaagtagtgaggaggcttttttggaggcctaggcttttgcaaaaagctcccgggagcttggatatccattttcggatctgatcaagagacaggatgaggatcgtttcgcatgattgaacaagatggattgcacgcaggttctccggccgcttgggtggagaggctattcggctatgactgggcacaacagacaatcggctgctctgatgccgccgtgttccggctgtcagcgcaggggcgcccggttctttttgtcaagaccgacctgtccggtgccctgaatgaactgcaggacgaggcagcgcggctatcgtggctggccacgacgggcgttccttgcgcagctgtgctcgacgttgtcactgaagcgggaagggactggctgctattgggcgaagtgccggggcaggatctcctgtcatctcaccttgctcctgccgagaaagtatccatcatggctgatgcaatgcggcggctgcatacgcttgatccggctacctgcccattcgaccaccaagcgaaacatcgcatcgagcgagcacgtactcggatggaagccggtcttgtcgatcaggatgatctggacgaagagcatcaggggctcgcgccagccgaactgttcgccaggctcaaggcgcgcatgcccgacggcgaggatctcgtcgtgacccatggcgatgcctgcttgccgaatatcatggtggaaaatggccgcttttctggattcatcgactgtggccggctgggtgtggcggaccgctatcaggacatagcgttggctacccgtgatattgctgaagagcttggcggcgaatgggctgaccgcttcctcgtgctttacggtatcgccgctcccgattcgcagcgcatcgccttctatcgccttcttgacgagttcttctgagcgggactctggggttcggtgctacgagatttcgattccaccgccgccttctatgaaaggttgggcttcggaatcgttttccgggacgccggctggatgatcctccagcgcggggatctcatgctggagttcttcgcccaccccaacttgtttattgcagcttataatggttacaaataaagcaatagcatcacaaatttcacaaataaagcatttttttcactgcattctagttgtggtttgtccaaactcatcaatgtatcttatcatgtctgtataccgtcgacctctagctagagcttggcgtaatcatggtcatagctgtttcctgtgtgaaattgttatccgctcacaattccacacaacatacgagccggaagcataaagtgtaaagcctggggtgcctaatgagtgagctaactcacattaattgcgttgcgctcactgcccgctttccagtcgggaaacctgtcgtgccagaattgcatgaagaatctgcttagggttaggcgttttgcgctgcttcgctaggtggtcaatattggccattagccatattattcattggttatatagcataaatcaatattggctattggccattgcatacgttgtatccatatcataatatgtacatttatattggctcatgtccaacattaccgccatgttgacattgattattgactagttattaatagtaatcaattacggggtcattagttcatagcccatatatggagttccgcgttacataacttacggtaaatggcccgcctggctgaccgcccaacgacccccgcccattgacgtcaataatgacgtatgttcccatagtaacgccaatagggactttccattgacgtcaatgggtggagtatttacggtaaactgcccacttggcagtacatcaagtgtatcatatgccaagtacgccccctattgacgtcaatgacggtaaatggcccgcctggcattatgcccagtacatgaccttatgggactttcctacttggcagtacatctacgtattagtcatcgctattaccatggtgatgcggttttggcagtacatcaatgggcgtggatagcggtttgactcacggggatttccaagtctccaccccattgacgtcaatgggagtttgttttggcaccaaaatcaacgggactttccaaaatgtcgtaacaactccgccccattgacgcaaatgggcggtaggcgtgtacggtgggaggtctatataagcagagctcgtttagtgaaccgtcagatcgcctggagacgccatccacgctgttttgacctccatagaagacaccgggaccgatccagcctccgcggccgggaacggtgcattggaagcttggtaccggtgaattaggcgcgccgtcgaggttatcgatccgaccgacgcgttcgcgagaggccgcaattccctagccaccatggcatgccctggcttcctgtgggcacttgtgatctccacctgtcttgaattctccatggctgacatccagatgacccagtctccatcctccctgtctgcatctgtaggagacagagtcaccatcacttgccgggcaagtcagagcattagcagctacttaaattggtatcagcagaaaccagggaaagcccctaagctcctgatctatgctgcatccagtttgcaaagtggggtcccatcaaggttcagtggcagtggatctgggacagatttcactctcaccatcagcagtctgcaacctgaagattttgcaacttactactgtcaacagagttacagtacccctccaacgttcggccaagggaccaaggtggagatcaaacgtaagtgcactttgcggccgctaggaagaaactcaaaacatcaagattttaaatacgcttcttggtctccttgctataattatctgggataagcatgctgttttctgtctgtccctaacatgccctgtgattatccgcaaacaacacacccaagggcagaactttgttacttaaacaccatcctgtttgcttctttcctcaggaactgtggctgcaccatctgtcttcatcttcccgccatctgatgagcagttgaaatctggaactgcctctgttgtgtgcctgctgaataacttctatcccagagaggccaaagtacagtggaaggtggataacgccctccaatcgggtaactcccaggagagtgtcacagagcaggacagcaaggacagcacctacagcctcagcagcaccctgacgctgagcaaagcagactacgagaaacacaaagtctacgcctgcgaagtcacccatcagggcctgagctcgcccgtcacaaagagcttcaacaggggagagtgttaggtttaacggatccgagctcggtaccaagctcaagtttaaaccgctgatcagcctcgactgtgccttctagttgccagccatctgttgtttgcccctcccccgtgccttccttgaccctggaaggtgccactcccactgtcctttcctaataaaatgaggaaattgcatcgcattgtctgagtaggtgtcattctattctggggggtggggtggggcaggacagcaagggggaggattgggaagacaatagcaggcatgctggggatgcggtgggctctatggcttctgaggcggaaagaaccagctgcattaatgaatcggccaacgcgcggggagaggcggtttgcgtattgggcgctcttccgcttcctcgctcactgactcgctgcgctcggtcgttcggctgcggcgagcggtatcagctcactcaaaggcggtaatacggttatccacagaatcaggggataacgcaggaaagaacatgtgagcaaaaggccagcaaaaggccaggaaccgtaaaaaggccgcgttgctggcgtttttccataggctccgcccccctgacgagcatcacaaaaatcgacgctcaagtcagaggtggcgaaacccgacaggactataaagataccaggcgtttccccctggaagctccctcgtgcgctctcctgttccgaccctgccgcttaccggatacctgtccgcctttctcccttcgggaagcgtggcgctttctcatagctcacgctgtaggtatctcagttcggtgtaggtcgttcgctccaagctgggctgtgtgcacgaaccccccgttcagcccgaccgctgcgccttatccggtaactatcgtcttgagtccaacccggtaagacacgacttatcgccactggcagcagccactggtaacaggattagcagagcgaggtatgtaggcggtgctacagagttcttgaagtggtggcctaactacggctacactagaagaacagtatttggtatctgcgctctgctgaagccagttaccttcggaaaaagagttggtagctcttgatccggcaaacaaaccaccgctggtagcggtggtttttttgtttgcaagcagcagattacgcgcagaaaaaaaggatctcaagaagatcctttgatcttttctacggggtctgacgctcagtggaacgaaaactcacgttaagggattttggtcatgagattatcaaaaaggatcttcacctagatccttttaaattaaaaatgaagttttaaatcaatctaaagtatatatgagtaaacttggtctgacagttaccaatgcttaatcagtgaggcacctatctcagcgatctgtctatttcgttcatccatagttgcctgactccccgtcgtgtagataactacgatacgggagggcttaccatctggccccagtgctgcaatgataccgcgagacccacgctcaccggctccagatttatcagcaataaaccagccagccggaagggccgagcgcagaagtggtcctgcaactttatccgcctccatccagtctattaattgttgccgggaagctagagtaagtagttcgccagttaatagtttgcgcaacgttgttgccattgctacaggcatcgtggtgtcacgctcgtcgtttggtatggcttcattcagctccggttcccaacgatcaaggcgagttacatgatcccccatgttgtgcaaaaaagcggttagctccttcggtcctccgatcgttgtcagaagtaagttggccgcagtgttatcactcatggttatggcagcactgcataattctcttactgtcatgccatccgtaagatgcttttctgtgactggtgagtactcaaccaagtcattctgagaatagtgtatgcggcgaccgagttgctcttgcccggcgtcaatacgggataataccgcgccacatagcagaactttaaaagtgctcatcattggaaaacgttcttcggggcgaaaactctcaaggatcttaccgctgttgagatccagttcgatgtaacccactcgtgcacccaactgatcttcagcatcttttactttcaccagcgtttctgggtgagcaaaaacaggaaggcaaaatgccgcaaaaaagggaataagggcgacacggaaatgttgaatactca

SEQ ID NO: 100 - DNA, 8179 bp, Artificial
  pCAGGS-IgVK1-39 targeting vector
atccaggcgcggatcaataaaagatcattattttcaatagatctgtgtgttggttttttgtgtgccttgggggagggggaggccagaatgaggcgcggccaagggggagggggaggccagaatgaccttgggggagggggaggccagaatgaccttgggggagggggaggccagaatgaggcgcggatccggagaagttcctattccgaagttcctattcttcaaatagtataggaacttcgctcgagggatcggccattgaacaagatggattgcacgcaggttctccggccgcttgggtggagaggctattcggctatgactgggcacaacagacaatcggctgctctgatgccgccgtgttccggctgtcagcgcaggggcgcccggttctttttgtcaagaccgacctgtccggtgccctgaatgaactgcaggacgaggcagcgcggctatcgtggctggccacgacgggcgttccttgcgcagctgtgctcgacgttgtcactgaagcgggaagggactggctgctattgggcgaagtgccggggcaggatctcctgtcatctcaccttgctcctgccgagaaagtatccatcatggctgatgcaatgcggcggctgcatacgcttgatccggctacctgcccattcgaccaccaagcgaaacatcgcatcgagcgagcacgtactcggatggaagccggtcttgtcgatcaggatgatctggacgaagagcatcaggggctcgcgccagccgaactgttcgccaggctcaaggcgcgcatgcccgacggcgaggatctcgtcgtgacccatggcgatgcctgcttgccgaatatcatggtggaaaatggccgcttttctggattcatcgactgtggccggctgggtgtggcggaccgctatcaggacatagcgttggctacccgtgatattgctgaagagcttggcggcgaatgggctgaccgcttcctcgtgctttacggtatcgccgctcccgattcgcagcgcatcgccttctatcgccttcttgacgagttcttctgaggggatcgatccgctgtaagtctgcagaaattgatgatctattaaacaataaagatgtccactaaaatggaagtttttcctgtcatactttgttaagaagggtgagaacagagtacctacattttgaatggaaggattggagctacgggggtgggggtggggtgggattagataaatgcctgctctttactgaaggctctttactattgctttatgataatgtttcatagttggatatcataatttaaacaagcaaaaccaaattaagggccagctcattcctcccactcatgatctatagatctatagatctctcgtgggatcattgtttttctcttgattcccactttgtggttctaagtactgtggtttccaaatgtgtcagtttcatagcctgaagaacgagatcagcagcctctgttccacatacacttcattctcagtattgttttgccaagttctaattccatcagaagctgactctagatggcgcgtatgcaggttttcgacattgattattgactagttattaatagtaatcaattacggggtcattagttcatagcccatatatggagttccgcgttacataacttacggtaaatggcccgcctggctgaccgcccaacgacccccgcccattgacgtcaataatgacgtatgttcccatagtaacgccaatagggactttccattgacgtcaatgggtggagtatttacggtaaactgcccacttggcagtacatcaagtgtatcatatgccaagtacgccccctattgacgtcaatgacggtaaatggcccgcctggcattatgcccagtacatgaccttatgggactttcctacttggcagtacatctacgtattagtcatcgctattaccatggtcgaggtgagccccacgttctgcttcactctccccatctcccccccctccccacccccaattttgtatttatttattttttaattattttgtgcagcgatgggggcggggggggggggggcgcgcgccaggcggggcggggcggggcgaggggcggggcggggcgaggcggagaggtgcggcggcagccaatcagagcggcgcgctccgaaagtttccttttatggcgaggcggcggcggcggcggccctataaaaagcgaagcgcgcggcgggcgggagtcgctgcgttgccttcgccccgtgccccgctccgcgccgcctcgcgccgcccgccccggctctgactgaccgcgttactcccacaggtgagcgggcgggacggcccttctcctccgggctgtaattagcgcttggtttaatgacggctcgtttcttttctgtggctgcgtgaaagccttaaagggctccgggagggccctttgtgcgggggggagcggctcggggggtgcgtgcgtgtgtgtgtgcgtggggagcgccgcgtgcggcccgcgctgcccggcggctgtgagcgctgcgggcgcggcgcggggctttgtgcgctccgcgtgtgcgcgaggggagcgcggccgggggcggtgccccgcggtgcgggggggctgcgaggggaacaaaggctgcgtgcggggtgtgtgcgtgggggggtgagcagggggtgtgggcgcggcggtcgggctgtaacccccccctgcacccccctccccgagttgctgagcacggcccggcttcgggtgcggggctccgtgcggggcgtggcgcggggctcgccgtgccgggcggggggtggcggcaggtgggggtgccgggcggggcggggccgcctcgggccggggagggctcgggggaggggcgcggcggccccggagcgccggcggctgtcgaggcgcggcgagccgcagccattgccttttatggtaatcgtgcgagagggcgcagggacttcctttgtcccaaatctgtgcggagccgaaatctgggaggcgccgccgcaccccctctagcgggcgcggggcgaagcggtgcggcgccggcaggaaggaaatgggcggggagggccttcgtgcgtcgccgcgccgccgtccccttctccctctccagcctcggggctgtccgcggggggacggctgccttcgggggggacggggcagggcggggttcggcttctggcgtgtgaccggcggctctagaagcgttggggtgagtactccctctcaaaagcgggcatgacttctgcgctaagattgtcagtttccaaaaacgaggaggatttgatattcacctggcccgcggtgatgcctttgagggtggccgcgtccatctggtcagaaaagacaatctttttgttgtcaagcttgaggtgtggcaggcttgagatctggccatacacttgagtgacattgacatccactttgcctttctctccacaggtgtccactcccagggcggcctccggagcgatcgccgatccgcctaggcaattgtttaaatcggccggccataacttcgtataatgtatgctatacgaagttatggatcctcacagtaggtggcatcgttcctttctgactgcccgccccccgcatgccgtcccgcgatattgagctccgaacctctcgccctgccgccgccggtgctccgtcgccgccgcgccgccatggaatcgaagccaccatggatcttaccggaaaactcgacgcaagaaaaatcagagagatcctcataaaggtcaagaagggcggaaagatcgccgtgtaattctagaccggttcgagatccaggcgcggatcaataaaagatcattattttcaatagatctgtgtgttggttttttgtgtgccttgggggagggggaggccagaatgaggcgcggccaagggggagggggaggccagaatgaccttgggggagggggaggccagaatgaccttgggggagggggaggccagaatgaggcgcgccctccgtcgacctataacttcgtataatgtatgctatacgaagttatggcggccgccaccatggacatgagagtgcccgcccagctcctggggctcctgctactctggctccgaggtaaggatggagaacactaggaatttactcagccagtgtgctcagtactgactggaacttcagggaagttctctgataacatgattaatagtaagaatatttgtttttatgtttccaatctcaggtgccagatgtgacatccagatgacccagagccccagcagcctgagcgccagcgtgggcgacagagtgaccatcacctgcagagccagccagagcatcagcagctacctgaactggtatcagcagaagcccggcaaggcccccaagctgctgatctacgccgccagctccctgcagagcggcgtgcccagcagattcagcggcagcggctccggcaccgacttcaccctgaccatcagcagcctgcagcccgaggacttcgccacctactactgccagcagagctacagcaccccccccaccttcggccagggcaccaaggtggagatcaagagagccgacgccgctcccaccgtgtccatcttcccccccagcatggaacagctgacctctggcggagccaccgtggtctgcttcgtgaacaacttctaccccagagacatcagcgtgaagtggaagatcgacggcagcgagcagagggacggcgtgctggacagcgtgaccgaccaggacagcaaggactccacctacagcatgagcagcaccctgagcctgaccaaggtggagtacgagaggcacaacctgtacacctgcgaggtggtgcacaagaccagctccagccccgtggtcaagtccttcaaccggaacgagtgttgagctagcttaagatttaaataggccggccgcgtcgacctcgagatccaggcgcggatcaataaaagatcattattttcaatagatctgtgtgttggttttttgtgtgccttgggggagggggaggccagaatgaggcgcggccaagggggagggggaggccagaatgaccttgggggagggggaggccagaatgaccttgggggagggggaggccagaatgaggcgcgcccccgggtaccgagctcgaattagtggatcctcacagtaggtggcatcgttcctttctgactgcccgccccccgcatgccgtcccgcgatattgagctccgaacctctcgccctgccgccgccggtgctccgtcgccgccgcgccgccatggaatcgcgccggtaaccgaagttcctatactttctagagaataggaacttcggaataggaacttcaagccggtacccagcttttgttccctttagtgagggttaatttcgagcttggcgtaatcatggtcatagctgtttcctgtgtgaaattgttatccgctcacaattccacacaacatacgagccgggagcataaagtgtaaagcctggggtgcctaatgagtgagctaactcacattaattgcgttgcgctcactgcccgctttccagtcgggaaacctgtcgtgccagctgcattaatgaatcggccaacgcgcggggagaggcggtttgcgtattgggcgctcttccgcttcctcgctcactgactcgctgcgctcggtcgttcggctgcggcgagcggtatcagctcactcaaaggcggtaatacggttatccacagaatcaggggataacgcaggaaagaacatgtgagcaaaaggccagcaaaaggccaggaaccgtaaaaaggccgcgttgctggcgtttttccataggctccgcccccctgacgagcatcacaaaaatcgacgctcaagtcagaggtggcgaaacccgacaggactataaagataccaggcgtttccccctggaagctccctcgtgcgctctcctgttccgaccctgccgcttaccggatacctgtccgcctttctcccttcgggaagcgtggcgctttctcatagctcacgctgtaggtatctcagttcggtgtaggtcgttcgctccaagctgggctgtgtgcacgaaccccccgttcagcccgaccgctgcgccttatccggtaactatcgtcttgagtccaacccggtaagacacgacttatcgccactggcagcagccactggtaacaggattagcagagcgaggtatgtaggcggtgctacagagttcttgaagtggtggcctaactacggctacactagaaggacagtatttggtatctgcgctctgctgaagccagttaccttcggaaaaagagttggtagctcttgatccggcaaacaaaccaccgctggtagcggtggtttttttgtttgcaagcagcagattacgcgcagaaaaaaaggatctcaagaagatcctttgatcttttctacggggtctgacgctcagtggaacgaaaactcacgttaagggattttggtcatgagattatcaaaaaggatcttcacctagatccttttaaattaaaaatgaagttttaaatcaatctaaagtatatatgagtaaacttggtctgacagttaccaatgcttaatcagtgaggcacctatctcagcgatctgtctatttcgttcatccatagttgcctgactccccgtcgtgtagataactacgatacgggagggcttaccatctggccccagtgctgcaatgataccgcgagacccacgctcaccggctccagatttatcagcaataaaccagccagccggaagggccgagcgcagaagtggtcctgcaactttatccgcctccatccagtctattaattgttgccgggaagctagagtaagtagttcgccagttaatagtttgcgcaacgttgttgccattgctacaggcatcgtggtgtcacgctcgtcgtttggtatggcttcattcagctccggttcccaacgatcaaggcgagttacatgatcccccatgttgtgcaaaaaagcggttagctccttcggtcctccgatcgttgtcagaagtaagttggccgcagtgttatcactcatggttatggcagcactgcataattctcttactgtcatgccatccgtaagatgcttttctgtgactggtgagtactcaaccaagtcattctgagaatagtgtatgcggcgaccgagttgctcttgcccggcgtcaatacgggataataccgcgccacatagcagaactttaaaagtgctcatcattggaaaacgttcttcggggcgaaaactctcaaggatcttaccgctgttgagatccagttcgatgtaacccactcgtgcacccaactgatcttcagcatcttttactttcaccagcgtttctgggtgagcaaaaacaggaaggcaaaatgccgcaaaaaagggaataagggcgacacggaaatgttgaatactcatactcttcctttttcaatattattgaagcatttatcagggttattgtctcatgagcggatacatatttgaatgtatttagaaaaataaacaaataggggttccgcgcacatttccccgaaaagtgccacctaaattgtaagcgttaatattttgttaaaattcgcgttaaatttttgttaaatcagctcattttttaaccaataggccgaaatcggcaaaatcccttataaatcaaaagaatagaccgagatagggttgagtgttgttccagtttggaacaagagtccactattaaagaacgtggactccaacgtcaaagggcgaaaaaccgtctatcagggcgatggcccactacgtgaaccatcaccctaatcaagttttttggggtcgaggtgccgtaaagcactaaatcggaaccctaaagggagcccccgatttagagcttgacggggaaagccggcgaacgtggcgagaaaggaagggaagaaagcgaaaggagcgggcgctagggcgctggcaagtgtagcggtcacgctgcgcgtaaccaccacacccgccgcgcttaatgcgccgctacagggcgcgtcccattcgccattcaggctgcgcaactgttgggaagggcgatcggtgcgggcctcttcgctattacgccagctggcgaaagggggatgtgctgcaaggcgattaagttgggtaacgccagggttttcccagtcacgacgttgtaaaacgacggccagtgagcgcgcgtaatacgactcactatagggcgaattgggggtaactaagtaaggatcgag

SEQ ID NO: 101 - DNA, 8188 bp, pCAGGS-IgVL2-14 targeting vector
atccaggcgcggatcaataaaagatcattattttcaatagatctgtgtgttggttttttgtgtgccttgggggagggggaggccagaatgaggcgcggccaagggggagggggaggccagaatgaccttgggggagggggaggccagaatgaccttgggggagggggaggccagaatgaggcgcggatccggagaagttcctattccgaagttcctattcttcaaatagtataggaacttcgctcgagggatcggccattgaacaagatggattgcacgcaggttctccggccgcttgggtggagaggctattcggctatgactgggcacaacagacaatcggctgctctgatgccgccgtgttccggctgtcagcgcaggggcgcccggttctttttgtcaagaccgacctgtccggtgccctgaatgaactgcaggacgaggcagcgcggctatcgtggctggccacgacgggcgttccttgcgcagctgtgctcgacgttgtcactgaagcgggaagggactggctgctattgggcgaagtgccggggcaggatctcctgtcatctcaccttgctcctgccgagaaagtatccatcatggctgatgcaatgcggcggctgcatacgcttgatccggctacctgcccattcgaccaccaagcgaaacatcgcatcgagcgagcacgtactcggatggaagccggtcttgtcgatcaggatgatctggacgaagagcatcaggggctcgcgccagccgaactgttcgccaggctcaaggcgcgcatgcccgacggcgaggatctcgtcgtgacccatggcgatgcctgcttgccgaatatcatggtggaaaatggccgcttttctggattcatcgactgtggccggctgggtgtggcggaccgctatcaggacatagcgttggctacccgtgatattgctgaagagcttggcggcgaatgggctgaccgcttcctcgtgctttacggtatcgccgctcccgattcgcagcgcatcgccttctatcgccttcttgacgagttcttctgaggggatcgatccgctgtaagtctgcagaaattgatgatctattaaacaataaagatgtccactaaaatggaagtttttcctgtcatactttgttaagaagggtgagaacagagtacctacattttgaatggaaggattggagctacgggggtgggggtggggtgggattagataaatgcctgctctttactgaaggctctttactattgctttatgataatgtttcatagttggatatcataatttaaacaagcaaaaccaaattaagggccagctcattcctcccactcatgatctatagatctatagatctctcgtgggatcattgtttttctcttgattcccactttgtggttctaagtactgtggtttccaaatgtgtcagtttcatagcctgaagaacgagatcagcagcctctgttccacatacacttcattctcagtattgttttgccaagttctaattccatcagaagctgactctagatggcgcgtatgcaggttttcgacattgattattgactagttattaatagtaatcaattacggggtcattagttcatagcccatatatggagttccgcgttacataacttacggtaaatggcccgcctggctgaccgcccaacgacccccgcccattgacgtcaataatgacgtatgttcccatagtaacgccaatagggactttccattgacgtcaatgggtggagtatttacggtaaactgcccacttggcagtacatcaagtgtatcatatgccaagtacgccccctattgacgtcaatgacggtaaatggcccgcctggcattatgcccagtacatgaccttatgggactttcctacttggcagtacatctacgtattagtcatcgctattaccatggtcgaggtgagccccacgttctgcttcactctccccatctcccccccctccccacccccaattttgtatttatttattttttaattattttgtgcagcgatgggggcggggggggggggggcgcgcgccaggcggggcggggcggggcgaggggcggggcggggcgaggcggagaggtgcggcggcagccaatcagagcggcgcgctccgaaagtttccttttatggcgaggcggcggcggcggcggccctataaaaagcgaagcgcgcggcgggcgggagtcgctgcgttgccttcgccccgtgccccgctccgcgccgcctcgcgccgcccgccccggctctgactgaccgcgttactcccacaggtgagcgggcgggacggcccttctcctccgggctgtaattagcgcttggtttaatgacggctcgtttcttttctgtggctgcgtgaaagccttaaagggctccgggagggccctttgtgcgggggggagcggctcggggggtgcgtgcgtgtgtgtgtgcgtggggagcgccgcgtgcggcccgcgctgcccggcggctgtgagcgctgcgggcgcggcgcggggctttgtgcgctccgcgtgtgcgcgaggggagcgcggccgggggcggtgccccgcggtgcgggggggctgcgaggggaacaaaggctgcgtgcggggtgtgtgcgtgggggggtgagcagggggtgtgggcgcggcggtcgggctgtaacccccccctgcacccccctccccgagttgctgagcacggcccggcttcgggtgcggggctccgtgcggggcgtggcgcggggctcgccgtgccgggcggggggtggcggcaggtgggggtgccgggcggggcggggccgcctcgggccggggagggctcgggggaggggcgcggcggccccggagcgccggcggctgtcgaggcgcggcgagccgcagccattgccttttatggtaatcgtgcgagagggcgcagggacttcctttgtcccaaatctgtgcggagccgaaatctgggaggcgccgccgcaccccctctagcgggcgcggggcgaagcggtgcggcgccggcaggaaggaaatgggcggggagggccttcgtgcgtcgccgcgccgccgtccccttctccctctccagcctcggggctgtccgcggggggacggctgccttcgggggggacggggcagggcggggttcggcttctggcgtgtgaccggcggctctagaagcgttggggtgagtactccctctcaaaagcgggcatgacttctgcgctaagattgtcagtttccaaaaacgaggaggatttgatattcacctggcccgcggtgatgcctttgagggtggccgcgtccatctggtcagaaaagacaatctttttgttgtcaagcttgaggtgtggcaggcttgagatctggccatacacttgagtgacattgacatccactttgcctttctctccacaggtgtccactcccagggcggcctccggagcgatcgccgatccgcctaggcaattgtttaaatcggccggccataacttcgtataatgtatgctatacgaagttatggatcctcacagtaggtggcatcgttcctttctgactgcccgccccccgcatgccgtcccgcgatattgagctccgaacctctcgccctgccgccgccggtgctccgtcgccgccgcgccgccatggaatcgaagccaccatggatcttaccggaaaactcgacgcaagaaaaatcagagagatcctcataaaggtcaagaagggcggaaagatcgccgtgtaattctagaccggttcgagatccaggcgcggatcaataaaagatcattattttcaatagatctgtgtgttggttttttgtgtgccttgggggagggggaggccagaatgaggcgcggccaagggggagggggaggccagaatgaccttgggggagggggaggccagaatgaccttgggggagggggaggccagaatgaggcgcgccctccgtcgacctataacttcgtataatgtatgctatacgaagttatggcggccgccaccatggacatgagagtgcccgcccagctcctggggctcctgctactctggctccgaggtaaggatggagaacactaggaatttactcagccagtgtgctcagtactgactggaacttcagggaagttctctgataacatgattaatagtaagaatatttgtttttatgtttccaatctcaggtgccagatgtcagtctgccctgacccagcccgcctctgtgtctggcagccctggccagagcatcaccatcagctgcaccggcaccagcagcgacgtgggcggctacaactacgtgtcctggtatcagcagcaccccggcaaggcccccaagctgatgatctacgaggtgtccaacagacccagcggcgtgagcaacagattcagcggcagcaagagcggcaacaccgccagcctgaccatcagcggcctccaggctgaggacgaggccgactactactgcagcagctacaccagcagctccaccctggtgtttggcggcggaacaaagctgaccgtgctgagagccgacgccgctcccaccgtgtccatcttcccccccagcatggaacagctgacctctggcggagccaccgtggtctgcttcgtgaacaacttctaccccagagacatcagcgtgaagtggaagatcgacggcagcgagcagagggacggcgtgctggacagcgtgaccgaccaggacagcaaggactccacctacagcatgagcagcaccctgagcctgaccaaggtggagtacgagaggcacaacctgtacacctgcgaggtggtgcacaagaccagctccagccccgtggtcaagtccttcaaccggaacgagtgttgagctagcttaagatttaaataggccggccgcgtcgacctcgagatccaggcgcggatcaataaaagatcattattttcaatagatctgtgtgttggttttttgtgtgccttgggggagggggaggccagaatgaggcgcggccaagggggagggggaggccagaatgaccttgggggagggggaggccagaatgaccttgggggagggggaggccagaatgaggcgcgcccccgggtaccgagctcgaattagtggatcctcacagtaggtggcatcgttcctttctgactgcccgccccccgcatgccgtcccgcgatattgagctccgaacctctcgccctgccgccgccggtgctccgtcgccgccgcgccgccatggaatcgcgccggtaaccgaagttcctatactttctagagaataggaacttcggaataggaacttcaagccggtacccagcttttgttccctttagtgagggttaatttcgagcttggcgtaatcatggtcatagctgtttcctgtgtgaaattgttatccgctcacaattccacacaacatacgagccgggagcataaagtgtaaagcctggggtgcctaatgagtgagctaactcacattaattgcgttgcgctcactgcccgctttccagtcgggaaacctgtcgtgccagctgcattaatgaatcggccaacgcgcggggagaggcggtttgcgtattgggcgctcttccgcttcctcgctcactgactcgctgcgctcggtcgttcggctgcggcgagcggtatcagctcactcaaaggcggtaatacggttatccacagaatcaggggataacgcaggaaagaacatgtgagcaaaaggccagcaaaaggccaggaaccgtaaaaaggccgcgttgctggcgtttttccataggctccgcccccctgacgagcatcacaaaaatcgacgctcaagtcagaggtggcgaaacccgacaggactataaagataccaggcgtttccccctggaagctccctcgtgcgctctcctgttccgaccctgccgcttaccggatacctgtccgcctttctcccttcgggaagcgtggcgctttctcatagctcacgctgtaggtatctcagttcggtgtaggtcgttcgctccaagctgggctgtgtgcacgaaccccccgttcagcccgaccgctgcgccttatccggtaactatcgtcttgagtccaacccggtaagacacgacttatcgccactggcagcagccactggtaacaggattagcagagcgaggtatgtaggcggtgctacagagttcttgaagtggtggcctaactacggctacactagaaggacagtatttggtatctgcgctctgctgaagccagttaccttcggaaaaagagttggtagctcttgatccggcaaacaaaccaccgctggtagcggtggtttttttgtttgcaagcagcagattacgcgcagaaaaaaaggatctcaagaagatcctttgatcttttctacggggtctgacgctcagtggaacgaaaactcacgttaagggattttggtcatgagattatcaaaaaggatcttcacctagatccttttaaattaaaaatgaagttttaaatcaatctaaagtatatatgagtaaacttggtctgacagttaccaatgcttaatcagtgaggcacctatctcagcgatctgtctatttcgttcatccatagttgcctgactccccgtcgtgtagataactacgatacgggagggcttaccatctggccccagtgctgcaatgataccgcgagacccacgctcaccggctccagatttatcagcaataaaccagccagccggaagggccgagcgcagaagtggtcctgcaactttatccgcctccatccagtctattaattgttgccgggaagctagagtaagtagttcgccagttaatagtttgcgcaacgttgttgccattgctacaggcatcgtggtgtcacgctcgtcgtttggtatggcttcattcagctccggttcccaacgatcaaggcgagttacatgatcccccatgttgtgcaaaaaagcggttagctccttcggtcctccgatcgttgtcagaagtaagttggccgcagtgttatcactcatggttatggcagcactgcataattctcttactgtcatgccatccgtaagatgcttttctgtgactggtgagtactcaaccaagtcattctgagaatagtgtatgcggcgaccgagttgctcttgcccggcgtcaatacgggataataccgcgccacatagcagaactttaaaagtgctcatcattggaaaacgttcttcggggcgaaaactctcaaggatcttaccgctgttgagatccagttcgatgtaacccactcgtgcacccaactgatcttcagcatcttttactttcaccagcgtttctgggtgagcaaaaacaggaaggcaaaatgccgcaaaaaagggaataagggcgacacggaaatgttgaatactcatactcttcctttttcaatattattgaagcatttatcagggttattgtctcatgagcggatacatatttgaatgtatttagaaaaataaacaaataggggttccgcgcacatttccccgaaaagtgccacctaaattgtaagcgttaatattttgttaaaattcgcgttaaatttttgttaaatcagctcattttttaaccaataggccgaaatcggcaaaatcccttataaatcaaaagaatagaccgagatagggttgagtgttgttccagtttggaacaagagtccactattaaagaacgtggactccaacgtcaaagggcgaaaaaccgtctatcagggcgatggcccactacgtgaaccatcaccctaatcaagttttttggggtcgaggtgccgtaaagcactaaatcggaaccctaaagggagcccccgatttagagcttgacggggaaagccggcgaacgtggcgagaaaggaagggaagaaagcgaaaggagcgggcgctagggcgctggcaagtgtagcggtcacgctgcgcgtaaccaccacacccgccgcgcttaatgcgccgctacagggcgcgtcccattcgccattcaggctgcgcaactgttgggaagggcgatcggtgcgggcctcttcgctattacgccagctggcgaaagggggatgtgctgcaaggcgattaagttgggtaacgccagggttttcccagtcacgacgttgtaaaacgacggccagtgagcgcgcgtaatacgactcactatagggcgaattgggggtaactaagtaaggatcgag